European Patent Application EP 4 810 057 A1, published September 23, 2026. Title: RSV疫苗组合物、方法及其用途. Applicant: 四川三叶草生物制 药有限公司. Application CN. The sequence listing filed with the application follows.

SEQUENCE LISTING (148 sequences)

SEQ ID NO: 1 - protein, 831 aa, synthetic construct
MELLILKANAITTILTAVTFCFASGQNITEEFYQSTCSAVSKGYLSALRTGWYTSVITIELSNIKENKCNGTDAKVKLIKQELDKYKNAVTELQLLMQSTPATNNRARRELPRFMNYTLNNAKKTNVTLSKKRKRRFLGFLLGVGSAIASGVAVSKVLHLEGEVNKIKSALLSTNKAVVSLSNGVSVLTSKVLDLKNYIDKQLLPIVNKQSCSISNIATVIEFQQKNNRLLEITREFSVNAGVTTPVSTYMLTNSELLSLINDMPITNDQKKLMSNNVQIVRQQSYSIMSIIKEEVLAYVVQLPLYGVIDTPCWKLHTSPLCTTNTKEGSNICLTRTDRGWYCDNAGSVSFFPQAETCKVQSNRVFCDTMNSLTLPSEVNLCNVDIFNPKYDCKIMTSKTDVSSSVITSLGAIVSCYGKTKCTASNKNRGIIKTFSNGCDYVSNKGVDTVSVGNTLYYVNKQEGKSLYVKGEPIINFYDPLVFPSDEFDASISQVNEKINQSLAFIRKSDELLHNVNAGKRSNGLPGPIGPPGPRGRTGDAGPVGPPGPPGPPGPPGPPSAGFDFSFLPQPPQEKAHDGGRYYRANDANVVRDRDLEVDTTLKSLSQQIENIRSPEGSRKNPARTCRDLKMCHSDWKSGEYWIDPNQGCNLDAIKVFCNMETGETCVYPTQPSVAQKNWYISKNPKDKRHVWFGESMTDGFQFEYGGQGSDPADVAIQLTFLRLMSTEASQNITYHCKNSVAYMDQQTGNLKKALLLQGSNEIEIRAEGNSRFTYSVTVDGCTSHTGAWGKTVIEYKTTKTSRLPIIDVAPLDVGAPDQEFGFDVGPVCFL

SEQ ID NO: 2 - protein, 831 aa, synthetic construct
MELLILKANAITTILTAVTFCFASGQNITEEFYQSTCSAVSKGYLSALRTGWYTSVITIELSNIKENKCNGTDAKVKLIKQELDKYKNAVTELQLLMQSTPATNNCACRELPRFMNYTLNNAKKTNVTLSKKCKCCFLGFLLGVGSAIASGVAVSKVLHLEGEVNKIKSALLSTNKAVVSLSNGVSVLTSKVLDLKNYIDKQLLPIVNKQSCSISNIATVIEFQQKNNRLLEITREFSVNAGVTTPVSTYMLTNSELLSLINDMPITNDQKKLMSNNVQIVRQQSYSIMSIIKEEVLAYVVQLPLYGVIDTPCWKLHTSPLCTTNTKEGSNICLTRTDRGWYCDNAGSVSFFPQAETCKVQSNRVFCDTMNSLTLPSEVNLCNVDIFNPKYDCKIMTSKTDVSSSVITSLGAIVSCYGKTKCTASNKNRGIIKTFSNGCDYVSNKGVDTVSVGNTLYYVNKQEGKSLYVKGEPIINFYDPLVFPSDEFDASISQVNEKINQSLAFIRKSDELLHNVNAGKRSNGLPGPIGPPGPRGRTGDAGPVGPPGPPGPPGPPGPPSAGFDFSFLPQPPQEKAHDGGRYYRANDANVVRDRDLEVDTTLKSLSQQIENIRSPEGSRKNPARTCRDLKMCHSDWKSGEYWIDPNQGCNLDAIKVFCNMETGETCVYPTQPSVAQKNWYISKNPKDKRHVWFGESMTDGFQFEYGGQGSDPADVAIQLTFLRLMSTEASQNITYHCKNSVAYMDQQTGNLKKALLLQGSNEIEIRAEGNSRFTYSVTVDGCTSHTGAWGKTVIEYKTTKTSRLPIIDVAPLDVGAPDQEFGFDVGPVCFL

SEQ ID NO: 3 - protein, 830 aa, synthetic construct
MELLILKANAITTILTAVTFCFASGQNITEEFYQSTCSAVSKGYLSALRTGWYTSVITIELSNIKENKCNGTDAKVKLIKQELDKYKNAVTELQLLMQSTPATNNRACRELPRFMNYTLNNAKKTNVTLSKKCKCCFLGFLLGVGSAIASGVAVSKVLHLEGEVNKIKSALLSTNKAVVSLSNGVSVLTSKVLDLKNYIDKQLLPIVNKQSCSISNIATVIEFQQKNNRLLEITREFSVNAGVTTPVSTYMLTNSELLSLINDMPITNDQKKLMSNNVQIVRQQSYSIMSIIKEEVLAYVVQLPLYGVIDTPCWKLHTSPLCTTNTKEGSNICLTRTDRGWYCDNAGSVSFFPQAETCKVQSNRVFCDTMNSLTLPSEVNLCNVDIFNPKYDCKIMTSKTDVSSSVITSLGAIVSCYGKTKCTASNKNRGIIKTFSNGCDYVSNKGVDTVSVGNTLYYVNKQEGKSLYVKGEPIINFYDPLVFPSDEFDASISQVNEKINQSLAFIRKSDELLHNVNAGKSNGLPGPIGPPGPRGRTGDAGPVGPPGPPGPPGPPGPPSAGFDFSFLPQPPQEKAHDGGRYYRANDANVVRDRDLEVDTTLKSLSQQIENIRSPEGSRKNPARTCRDLKMCHSDWKSGEYWIDPNQGCNLDAIKVFCNMETGETCVYPTQPSVAQKNWYISKNPKDKRHVWFGESMTDGFQFEYGGQGSDPADVAIQLTFLRLMSTEASQNITYHCKNSVAYMDQQTGNLKKALLLQGSNEIEIRAEGNSRFTYSVTVDGCTSHTGAWGKTVIEYKTTKTSRLPIIDVAPLDVGAPDQEFGFDVGPVCFL

SEQ ID NO: 4 - protein, 831 aa, synthetic construct
MELLILKANAITTILTAVTFCFASGQNITEEFYQSTCSAVSKGYLSALRTGWYTSVITIELSNIKENKCNGTDAKVKLIKQELDKYKNAVTELQLLMQSTPATNNRARRELPRFMNYTLNNAKKTNVTLSKKCKCCFLGFLLGVGSAIASGVAVSKVLHLEGEVNKIKSALLSTNKAVVSLSNGVSVLTSKVLDLKNYIDKQLLPIVNKQSCSISNIATVIEFQQKNNRLLEITREFSVNAGVTTPVSTYMLTNSELLSLINDMPITNDQKKLMSNNVQIVRQQSYSIMSIIKEEVLAYVVQLPLYGVIDTPCWKLHTSPLCTTNTKEGSNICLTRTDRGWYCDNAGSVSFFPQAETCKVQSNRVFCDTMNSLTLPSEVNLCNVDIFNPKYDCKIMTSKTDVSSSVITSLGAIVSCYGKTKCTASNKNRGIIKTFSNGCDYVSNKGVDTVSVGNTLYYVNKQEGKSLYVKGEPIINFYDPLVFPSDEFDASISQVNEKINQSLAFIRKSDELLHNVNAGKRSNGLPGPIGPPGPRGRTGDAGPVGPPGPPGPPGPPGPPSAGFDFSFLPQPPQEKAHDGGRYYRANDANVVRDRDLEVDTTLKSLSQQIENIRSPEGSRKNPARTCRDLKMCHSDWKSGEYWIDPNQGCNLDAIKVFCNMETGETCVYPTQPSVAQKNWYISKNPKDKRHVWFGESMTDGFQFEYGGQGSDPADVAIQLTFLRLMSTEASQNITYHCKNSVAYMDQQTGNLKKALLLQGSNEIEIRAEGNSRFTYSVTVDGCTSHTGAWGKTVIEYKTTKTSRLPIIDVAPLDVGAPDQEFGFDVGPVCFL

SEQ ID NO: 5 - protein, 831 aa, synthetic construct
MELLILKANAITTILTAVTFCFASGQNITEEFYQSTCSAVSKGYLSALRTGWYTSVITIELSNIKENKCNGTDAKVKLIKQELDKYKNAVTELQLLMQSTPATNNRARRELPRFMNYTLNNAKKTNVTLSKKRKCCFLGFLLGVGSAIASGVAVSKVLHLEGEVNKIKSALLSTNKAVVSLSNGVSVLTSKVLDLKNYIDKQLLPIVNKQSCSISNIATVIEFQQKNNRLLEITREFSVNAGVTTPVSTYMLTNSELLSLINDMPITNDQKKLMSNNVQIVRQQSYSIMSIIKEEVLAYVVQLPLYGVIDTPCWKLHTSPLCTTNTKEGSNICLTRTDRGWYCDNAGSVSFFPQAETCKVQSNRVFCDTMNSLTLPSEVNLCNVDIFNPKYDCKIMTSKTDVSSSVITSLGAIVSCYGKTKCTASNKNRGIIKTFSNGCDYVSNKGVDTVSVGNTLYYVNKQEGKSLYVKGEPIINFYDPLVFPSDEFDASISQVNEKINQSLAFIRKSDELLHNVNAGKRSNGLPGPIGPPGPRGRTGDAGPVGPPGPPGPPGPPGPPSAGFDFSFLPQPPQEKAHDGGRYYRANDANVVRDRDLEVDTTLKSLSQQIENIRSPEGSRKNPARTCRDLKMCHSDWKSGEYWIDPNQGCNLDAIKVFCNMETGETCVYPTQPSVAQKNWYISKNPKDKRHVWFGESMTDGFQFEYGGQGSDPADVAIQLTFLRLMSTEASQNITYHCKNSVAYMDQQTGNLKKALLLQGSNEIEIRAEGNSRFTYSVTVDGCTSHTGAWGKTVIEYKTTKTSRLPIIDVAPLDVGAPDQEFGFDVGPVCFL

SEQ ID NO: 6 - protein, 806 aa, synthetic construct
QNITEEFYQSTCSAVSKGYLSALRTGWYTSVITIELSNIKENKCNGTDAKVKLIKQELDKYKNAVTELQLLMQSTPATNNRARRELPRFMNYTLNNAKKTNVTLSKKRKRRFLGFLLGVGSAIASGVAVSKVLHLEGEVNKIKSALLSTNKAVVSLSNGVSVLTSKVLDLKNYIDKQLLPIVNKQSCSISNIATVIEFQQKNNRLLEITREFSVNAGVTTPVSTYMLTNSELLSLINDMPITNDQKKLMSNNVQIVRQQSYSIMSIIKEEVLAYVVQLPLYGVIDTPCWKLHTSPLCTTNTKEGSNICLTRTDRGWYCDNAGSVSFFPQAETCKVQSNRVFCDTMNSLTLPSEVNLCNVDIFNPKYDCKIMTSKTDVSSSVITSLGAIVSCYGKTKCTASNKNRGIIKTFSNGCDYVSNKGVDTVSVGNTLYYVNKQEGKSLYVKGEPIINFYDPLVFPSDEFDASISQVNEKINQSLAFIRKSDELLHNVNAGKRSNGLPGPIGPPGPRGRTGDAGPVGPPGPPGPPGPPGPPSAGFDFSFLPQPPQEKAHDGGRYYRANDANVVRDRDLEVDTTLKSLSQQIENIRSPEGSRKNPARTCRDLKMCHSDWKSGEYWIDPNQGCNLDAIKVFCNMETGETCVYPTQPSVAQKNWYISKNPKDKRHVWFGESMTDGFQFEYGGQGSDPADVAIQLTFLRLMSTEASQNITYHCKNSVAYMDQQTGNLKKALLLQGSNEIEIRAEGNSRFTYSVTVDGCTSHTGAWGKTVIEYKTTKTSRLPIIDVAPLDVGAPDQEFGFDVGPVCFL

SEQ ID NO: 7 - protein, 806 aa, synthetic construct
QNITEEFYQSTCSAVSKGYLSALRTGWYTSVITIELSNIKENKCNGTDAKVKLIKQELDKYKNAVTELQLLMQSTPATNNCACRELPRFMNYTLNNAKKTNVTLSKKCKCCFLGFLLGVGSAIASGVAVSKVLHLEGEVNKIKSALLSTNKAVVSLSNGVSVLTSKVLDLKNYIDKQLLPIVNKQSCSISNIATVIEFQQKNNRLLEITREFSVNAGVTTPVSTYMLTNSELLSLINDMPITNDQKKLMSNNVQIVRQQSYSIMSIIKEEVLAYVVQLPLYGVIDTPCWKLHTSPLCTTNTKEGSNICLTRTDRGWYCDNAGSVSFFPQAETCKVQSNRVFCDTMNSLTLPSEVNLCNVDIFNPKYDCKIMTSKTDVSSSVITSLGAIVSCYGKTKCTASNKNRGIIKTFSNGCDYVSNKGVDTVSVGNTLYYVNKQEGKSLYVKGEPIINFYDPLVFPSDEFDASISQVNEKINQSLAFIRKSDELLHNVNAGKRSNGLPGPIGPPGPRGRTGDAGPVGPPGPPGPPGPPGPPSAGFDFSFLPQPPQEKAHDGGRYYRANDANVVRDRDLEVDTTLKSLSQQIENIRSPEGSRKNPARTCRDLKMCHSDWKSGEYWIDPNQGCNLDAIKVFCNMETGETCVYPTQPSVAQKNWYISKNPKDKRHVWFGESMTDGFQFEYGGQGSDPADVAIQLTFLRLMSTEASQNITYHCKNSVAYMDQQTGNLKKALLLQGSNEIEIRAEGNSRFTYSVTVDGCTSHTGAWGKTVIEYKTTKTSRLPIIDVAPLDVGAPDQEFGFDVGPVCFL

SEQ ID NO: 8 - protein, 806 aa, synthetic construct
QNITEEFYQSTCSAVSKGYLSALRTGWYTSVITIELSNIKENKCNGTDAKVKLIKQELDKYKNAVTELQLLMQSTPATNNRACRELPRFMNYTLNNAKKTNVTLSKKCKCCFLGFLLGVGSAIASGVAVSKVLHLEGEVNKIKSALLSTNKAVVSLSNGVSVLTSKVLDLKNYIDKQLLPIVNKQSCSISNIATVIEFQQKNNRLLEITREFSVNAGVTTPVSTYMLTNSELLSLINDMPITNDQKKLMSNNVQIVRQQSYSIMSIIKEEVLAYVVQLPLYGVIDTPCWKLHTSPLCTTNTKEGSNICLTRTDRGWYCDNAGSVSFFPQAETCKVQSNRVFCDTMNSLTLPSEVNLCNVDIFNPKYDCKIMTSKTDVSSSVITSLGAIVSCYGKTKCTASNKNRGIIKTFSNGCDYVSNKGVDTVSVGNTLYYVNKQEGKSLYVKGEPIINFYDPLVFPSDEFDASISQVNEKINQSLAFIRKSDELLHNVNAGKRSNGLPGPIGPPGPRGRTGDAGPVGPPGPPGPPGPPGPPSAGFDFSFLPQPPQEKAHDGGRYYRANDANVVRDRDLEVDTTLKSLSQQIENIRSPEGSRKNPARTCRDLKMCHSDWKSGEYWIDPNQGCNLDAIKVFCNMETGETCVYPTQPSVAQKNWYISKNPKDKRHVWFGESMTDGFQFEYGGQGSDPADVAIQLTFLRLMSTEASQNITYHCKNSVAYMDQQTGNLKKALLLQGSNEIEIRAEGNSRFTYSVTVDGCTSHTGAWGKTVIEYKTTKTSRLPIIDVAPLDVGAPDQEFGFDVGPVCFL

SEQ ID NO: 9 - protein, 806 aa, synthetic construct
QNITEEFYQSTCSAVSKGYLSALRTGWYTSVITIELSNIKENKCNGTDAKVKLIKQELDKYKNAVTELQLLMQSTPATNNRARRELPRFMNYTLNNAKKTNVTLSKKCKCCFLGFLLGVGSAIASGVAVSKVLHLEGEVNKIKSALLSTNKAVVSLSNGVSVLTSKVLDLKNYIDKQLLPIVNKQSCSISNIATVIEFQQKNNRLLEITREFSVNAGVTTPVSTYMLTNSELLSLINDMPITNDQKKLMSNNVQIVRQQSYSIMSIIKEEVLAYVVQLPLYGVIDTPCWKLHTSPLCTTNTKEGSNICLTRTDRGWYCDNAGSVSFFPQAETCKVQSNRVFCDTMNSLTLPSEVNLCNVDIFNPKYDCKIMTSKTDVSSSVITSLGAIVSCYGKTKCTASNKNRGIIKTFSNGCDYVSNKGVDTVSVGNTLYYVNKQEGKSLYVKGEPIINFYDPLVFPSDEFDASISQVNEKINQSLAFIRKSDELLHNVNAGKRSNGLPGPIGPPGPRGRTGDAGPVGPPGPPGPPGPPGPPSAGFDFSFLPQPPQEKAHDGGRYYRANDANVVRDRDLEVDTTLKSLSQQIENIRSPEGSRKNPARTCRDLKMCHSDWKSGEYWIDPNQGCNLDAIKVFCNMETGETCVYPTQPSVAQKNWYISKNPKDKRHVWFGESMTDGFQFEYGGQGSDPADVAIQLTFLRLMSTEASQNITYHCKNSVAYMDQQTGNLKKALLLQGSNEIEIRAEGNSRFTYSVTVDGCTSHTGAWGKTVIEYKTTKTSRLPIIDVAPLDVGAPDQEFGFDVGPVCFL

SEQ ID NO: 10 - protein, 806 aa, synthetic construct
QNITEEFYQSTCSAVSKGYLSALRTGWYTSVITIELSNIKENKCNGTDAKVKLIKQELDKYKNAVTELQLLMQSTPATNNRARRELPRFMNYTLNNAKKTNVTLSKKRKCCFLGFLLGVGSAIASGVAVSKVLHLEGEVNKIKSALLSTNKAVVSLSNGVSVLTSKVLDLKNYIDKQLLPIVNKQSCSISNIATVIEFQQKNNRLLEITREFSVNAGVTTPVSTYMLTNSELLSLINDMPITNDQKKLMSNNVQIVRQQSYSIMSIIKEEVLAYVVQLPLYGVIDTPCWKLHTSPLCTTNTKEGSNICLTRTDRGWYCDNAGSVSFFPQAETCKVQSNRVFCDTMNSLTLPSEVNLCNVDIFNPKYDCKIMTSKTDVSSSVITSLGAIVSCYGKTKCTASNKNRGIIKTFSNGCDYVSNKGVDTVSVGNTLYYVNKQEGKSLYVKGEPIINFYDPLVFPSDEFDASISQVNEKINQSLAFIRKSDELLHNVNAGKRSNGLPGPIGPPGPRGRTGDAGPVGPPGPPGPPGPPGPPSAGFDFSFLPQPPQEKAHDGGRYYRANDANVVRDRDLEVDTTLKSLSQQIENIRSPEGSRKNPARTCRDLKMCHSDWKSGEYWIDPNQGCNLDAIKVFCNMETGETCVYPTQPSVAQKNWYISKNPKDKRHVWFGESMTDGFQFEYGGQGSDPADVAIQLTFLRLMSTEASQNITYHCKNSVAYMDQQTGNLKKALLLQGSNEIEIRAEGNSRFTYSVTVDGCTSHTGAWGKTVIEYKTTKTSRLPIIDVAPLDVGAPDQEFGFDVGPVCFL

SEQ ID NO: 11 - protein, 520 aa, synthetic construct
MELLILKANAITTILTAVTFCFASGQNITEEFYQSTCSAVSKGYLSALRTGWYTSVITIELSNIKENKCNGTDAKVKLIKQELDKYKNAVTELQLLMQSTPATNNRARRELPRFMNYTLNNAKKTNVTLSKKRKRRFLGFLLGVGSAIASGVAVSKVLHLEGEVNKIKSALLSTNKAVVSLSNGVSVLTSKVLDLKNYIDKQLLPIVNKQSCSISNIATVIEFQQKNNRLLEITREFSVNAGVTTPVSTYMLTNSELLSLINDMPITNDQKKLMSNNVQIVRQQSYSIMSIIKEEVLAYVVQLPLYGVIDTPCWKLHTSPLCTTNTKEGSNICLTRTDRGWYCDNAGSVSFFPQAETCKVQSNRVFCDTMNSLTLPSEVNLCNVDIFNPKYDCKIMTSKTDVSSSVITSLGAIVSCYGKTKCTASNKNRGIIKTFSNGCDYVSNKGVDTVSVGNTLYYVNKQEGKSLYVKGEPIINFYDPLVFPSDEFDASISQVNEKINQSLAFIRKSDELLHNVNAGK

SEQ ID NO: 12 - protein, 520 aa, synthetic construct
MELLILKANAITTILTAVTFCFASGQNITEEFYQSTCSAVSKGYLSALRTGWYTSVITIELSNIKENKCNGTDAKVKLIKQELDKYKNAVTELQLLMQSTPATNNCACRELPRFMNYTLNNAKKTNVTLSKKCKCCFLGFLLGVGSAIASGVAVSKVLHLEGEVNKIKSALLSTNKAVVSLSNGVSVLTSKVLDLKNYIDKQLLPIVNKQSCSISNIATVIEFQQKNNRLLEITREFSVNAGVTTPVSTYMLTNSELLSLINDMPITNDQKKLMSNNVQIVRQQSYSIMSIIKEEVLAYVVQLPLYGVIDTPCWKLHTSPLCTTNTKEGSNICLTRTDRGWYCDNAGSVSFFPQAETCKVQSNRVFCDTMNSLTLPSEVNLCNVDIFNPKYDCKIMTSKTDVSSSVITSLGAIVSCYGKTKCTASNKNRGIIKTFSNGCDYVSNKGVDTVSVGNTLYYVNKQEGKSLYVKGEPIINFYDPLVFPSDEFDASISQVNEKINQSLAFIRKSDELLHNVNAGK

SEQ ID NO: 13 - protein, 520 aa, synthetic construct
MELLILKANAITTILTAVTFCFASGQNITEEFYQSTCSAVSKGYLSALRTGWYTSVITIELSNIKENKCNGTDAKVKLIKQELDKYKNAVTELQLLMQSTPATNNRACRELPRFMNYTLNNAKKTNVTLSKKCKCCFLGFLLGVGSAIASGVAVSKVLHLEGEVNKIKSALLSTNKAVVSLSNGVSVLTSKVLDLKNYIDKQLLPIVNKQSCSISNIATVIEFQQKNNRLLEITREFSVNAGVTTPVSTYMLTNSELLSLINDMPITNDQKKLMSNNVQIVRQQSYSIMSIIKEEVLAYVVQLPLYGVIDTPCWKLHTSPLCTTNTKEGSNICLTRTDRGWYCDNAGSVSFFPQAETCKVQSNRVFCDTMNSLTLPSEVNLCNVDIFNPKYDCKIMTSKTDVSSSVITSLGAIVSCYGKTKCTASNKNRGIIKTFSNGCDYVSNKGVDTVSVGNTLYYVNKQEGKSLYVKGEPIINFYDPLVFPSDEFDASISQVNEKINQSLAFIRKSDELLHNVNAGK

SEQ ID NO: 14 - protein, 520 aa, synthetic construct
MELLILKANAITTILTAVTFCFASGQNITEEFYQSTCSAVSKGYLSALRTGWYTSVITIELSNIKENKCNGTDAKVKLIKQELDKYKNAVTELQLLMQSTPATNNRARRELPRFMNYTLNNAKKTNVTLSKKCKCCFLGFLLGVGSAIASGVAVSKVLHLEGEVNKIKSALLSTNKAVVSLSNGVSVLTSKVLDLKNYIDKQLLPIVNKQSCSISNIATVIEFQQKNNRLLEITREFSVNAGVTTPVSTYMLTNSELLSLINDMPITNDQKKLMSNNVQIVRQQSYSIMSIIKEEVLAYVVQLPLYGVIDTPCWKLHTSPLCTTNTKEGSNICLTRTDRGWYCDNAGSVSFFPQAETCKVQSNRVFCDTMNSLTLPSEVNLCNVDIFNPKYDCKIMTSKTDVSSSVITSLGAIVSCYGKTKCTASNKNRGIIKTFSNGCDYVSNKGVDTVSVGNTLYYVNKQEGKSLYVKGEPIINFYDPLVFPSDEFDASISQVNEKINQSLAFIRKSDELLHNVNAGK

SEQ ID NO: 15 - protein, 520 aa, synthetic construct
MELLILKANAITTILTAVTFCFASGQNITEEFYQSTCSAVSKGYLSALRTGWYTSVITIELSNIKENKCNGTDAKVKLIKQELDKYKNAVTELQLLMQSTPATNNRARRELPRFMNYTLNNAKKTNVTLSKKRKCCFLGFLLGVGSAIASGVAVSKVLHLEGEVNKIKSALLSTNKAVVSLSNGVSVLTSKVLDLKNYIDKQLLPIVNKQSCSISNIATVIEFQQKNNRLLEITREFSVNAGVTTPVSTYMLTNSELLSLINDMPITNDQKKLMSNNVQIVRQQSYSIMSIIKEEVLAYVVQLPLYGVIDTPCWKLHTSPLCTTNTKEGSNICLTRTDRGWYCDNAGSVSFFPQAETCKVQSNRVFCDTMNSLTLPSEVNLCNVDIFNPKYDCKIMTSKTDVSSSVITSLGAIVSCYGKTKCTASNKNRGIIKTFSNGCDYVSNKGVDTVSVGNTLYYVNKQEGKSLYVKGEPIINFYDPLVFPSDEFDASISQVNEKINQSLAFIRKSDELLHNVNAGK

SEQ ID NO: 16 - protein, 495 aa, synthetic construct
QNITEEFYQSTCSAVSKGYLSALRTGWYTSVITIELSNIKENKCNGTDAKVKLIKQELDKYKNAVTELQLLMQSTPATNNRARRELPRFMNYTLNNAKKTNVTLSKKRKRRFLGFLLGVGSAIASGVAVSKVLHLEGEVNKIKSALLSTNKAVVSLSNGVSVLTSKVLDLKNYIDKQLLPIVNKQSCSISNIATVIEFQQKNNRLLEITREFSVNAGVTTPVSTYMLTNSELLSLINDMPITNDQKKLMSNNVQIVRQQSYSIMSIIKEEVLAYVVQLPLYGVIDTPCWKLHTSPLCTTNTKEGSNICLTRTDRGWYCDNAGSVSFFPQAETCKVQSNRVFCDTMNSLTLPSEVNLCNVDIFNPKYDCKIMTSKTDVSSSVITSLGAIVSCYGKTKCTASNKNRGIIKTFSNGCDYVSNKGVDTVSVGNTLYYVNKQEGKSLYVKGEPIINFYDPLVFPSDEFDASISQVNEKINQSLAFIRKSDELLHNVNAGK

SEQ ID NO: 17 - protein, 495 aa, synthetic construct
QNITEEFYQSTCSAVSKGYLSALRTGWYTSVITIELSNIKENKCNGTDAKVKLIKQELDKYKNAVTELQLLMQSTPATNNCACRELPRFMNYTLNNAKKTNVTLSKKCKCCFLGFLLGVGSAIASGVAVSKVLHLEGEVNKIKSALLSTNKAVVSLSNGVSVLTSKVLDLKNYIDKQLLPIVNKQSCSISNIATVIEFQQKNNRLLEITREFSVNAGVTTPVSTYMLTNSELLSLINDMPITNDQKKLMSNNVQIVRQQSYSIMSIIKEEVLAYVVQLPLYGVIDTPCWKLHTSPLCTTNTKEGSNICLTRTDRGWYCDNAGSVSFFPQAETCKVQSNRVFCDTMNSLTLPSEVNLCNVDIFNPKYDCKIMTSKTDVSSSVITSLGAIVSCYGKTKCTASNKNRGIIKTFSNGCDYVSNKGVDTVSVGNTLYYVNKQEGKSLYVKGEPIINFYDPLVFPSDEFDASISQVNEKINQSLAFIRKSDELLHNVNAGK

SEQ ID NO: 18 - protein, 495 aa, synthetic construct
QNITEEFYQSTCSAVSKGYLSALRTGWYTSVITIELSNIKENKCNGTDAKVKLIKQELDKYKNAVTELQLLMQSTPATNNRACRELPRFMNYTLNNAKKTNVTLSKKCKCCFLGFLLGVGSAIASGVAVSKVLHLEGEVNKIKSALLSTNKAVVSLSNGVSVLTSKVLDLKNYIDKQLLPIVNKQSCSISNIATVIEFQQKNNRLLEITREFSVNAGVTTPVSTYMLTNSELLSLINDMPITNDQKKLMSNNVQIVRQQSYSIMSIIKEEVLAYVVQLPLYGVIDTPCWKLHTSPLCTTNTKEGSNICLTRTDRGWYCDNAGSVSFFPQAETCKVQSNRVFCDTMNSLTLPSEVNLCNVDIFNPKYDCKIMTSKTDVSSSVITSLGAIVSCYGKTKCTASNKNRGIIKTFSNGCDYVSNKGVDTVSVGNTLYYVNKQEGKSLYVKGEPIINFYDPLVFPSDEFDASISQVNEKINQSLAFIRKSDELLHNVNAGK

SEQ ID NO: 19 - protein, 495 aa, synthetic construct
QNITEEFYQSTCSAVSKGYLSALRTGWYTSVITIELSNIKENKCNGTDAKVKLIKQELDKYKNAVTELQLLMQSTPATNNRARRELPRFMNYTLNNAKKTNVTLSKKCKCCFLGFLLGVGSAIASGVAVSKVLHLEGEVNKIKSALLSTNKAVVSLSNGVSVLTSKVLDLKNYIDKQLLPIVNKQSCSISNIATVIEFQQKNNRLLEITREFSVNAGVTTPVSTYMLTNSELLSLINDMPITNDQKKLMSNNVQIVRQQSYSIMSIIKEEVLAYVVQLPLYGVIDTPCWKLHTSPLCTTNTKEGSNICLTRTDRGWYCDNAGSVSFFPQAETCKVQSNRVFCDTMNSLTLPSEVNLCNVDIFNPKYDCKIMTSKTDVSSSVITSLGAIVSCYGKTKCTASNKNRGIIKTFSNGCDYVSNKGVDTVSVGNTLYYVNKQEGKSLYVKGEPIINFYDPLVFPSDEFDASISQVNEKINQSLAFIRKSDELLHNVNAGK

SEQ ID NO: 20 - protein, 495 aa, synthetic construct
QNITEEFYQSTCSAVSKGYLSALRTGWYTSVITIELSNIKENKCNGTDAKVKLIKQELDKYKNAVTELQLLMQSTPATNNRARRELPRFMNYTLNNAKKTNVTLSKKRKCCFLGFLLGVGSAIASGVAVSKVLHLEGEVNKIKSALLSTNKAVVSLSNGVSVLTSKVLDLKNYIDKQLLPIVNKQSCSISNIATVIEFQQKNNRLLEITREFSVNAGVTTPVSTYMLTNSELLSLINDMPITNDQKKLMSNNVQIVRQQSYSIMSIIKEEVLAYVVQLPLYGVIDTPCWKLHTSPLCTTNTKEGSNICLTRTDRGWYCDNAGSVSFFPQAETCKVQSNRVFCDTMNSLTLPSEVNLCNVDIFNPKYDCKIMTSKTDVSSSVITSLGAIVSCYGKTKCTASNKNRGIIKTFSNGCDYVSNKGVDTVSVGNTLYYVNKQEGKSLYVKGEPIINFYDPLVFPSDEFDASISQVNEKINQSLAFIRKSDELLHNVNAGK

SEQ ID NO: 21 - protein, 831 aa, synthetic construct
MELLIHRSSAIFLTLAINALYLTSSQNITEEFYQSTCSAVSRGYLSALRTGWYTSVITIELSNIKETKCNGTDTKVKLIKQELDKYKNAVTELQLLMQNTPAVNNRARREAPQYMNYTINTTKNLNVSISKKRKRRFLGFLLGVGSAIASGIAVSKVLHLEGEVNKIKNALQLTNKAVVSLSNGVSVLTSRVLDLKNYINNQLLPMVNRQSCRISNIETVIEFQQKNSRLLEITREFSVNAGVTTPLSTYMLTNSELLSLINDMPITNDQKKLMSSNVQIVRQQSYSIMSIIKEEVLAYVVQLPIYGVIDTPCWKLHTSPLCTTNIKEGSNICLTRTDRGWYCDNAGSVSFFPQADTCKVQSNRVFCDTMNSLTLPSEVSLCNTDIFNSKYDCKIMTSKTDISSSVITSLGAIVSCYGKTKCTASNKNRGIIKTFSNGCDYVSNKGVDTVSVGNTLYYVNKLEGKNLYVKGEPIINYYDPLVFPSDEFDASISQVNEKINQSLAFIRRSDELLHNVNTGKRSNGLPGPIGPPGPRGRTGDAGPVGPPGPPGPPGPPGPPSAGFDFSFLPQPPQEKAHDGGRYYRANDANVVRDRDLEVDTTLKSLSQQIENIRSPEGSRKNPARTCRDLKMCHSDWKSGEYWIDPNQGCNLDAIKVFCNMETGETCVYPTQPSVAQKNWYISKNPKDKRHVWFGESMTDGFQFEYGGQGSDPADVAIQLTFLRLMSTEASQNITYHCKNSVAYMDQQTGNLKKALLLQGSNEIEIRAEGNSRFTYSVTVDGCTSHTGAWGKTVIEYKTTKTSRLPIIDVAPLDVGAPDQEFGFDVGPVCFL

SEQ ID NO: 22 - protein, 831 aa, synthetic construct
MELLIHRSSAIFLTLAINALYLTSSQNITEEFYQSTCSAVSRGYLSALRTGWYTSVITIELSNIKETKCNGTDTKVKLIKQELDKYKNAVTELQLLMQNTPAVNNCACREAPQYMNYTINTTKNLNVSISKKCKCCFLGFLLGVGSAIASGIAVSKVLHLEGEVNKIKNALQLTNKAVVSLSNGVSVLTSRVLDLKNYINNQLLPMVNRQSCRISNIETVIEFQQKNSRLLEITREFSVNAGVTTPLSTYMLTNSELLSLINDMPITNDQKKLMSSNVQIVRQQSYSIMSIIKEEVLAYVVQLPIYGVIDTPCWKLHTSPLCTTNIKEGSNICLTRTDRGWYCDNAGSVSFFPQADTCKVQSNRVFCDTMNSLTLPSEVSLCNTDIFNSKYDCKIMTSKTDISSSVITSLGAIVSCYGKTKCTASNKNRGIIKTFSNGCDYVSNKGVDTVSVGNTLYYVNKLEGKNLYVKGEPIINYYDPLVFPSDEFDASISQVNEKINQSLAFIRRSDELLHNVNTGKRSNGLPGPIGPPGPRGRTGDAGPVGPPGPPGPPGPPGPPSAGFDFSFLPQPPQEKAHDGGRYYRANDANVVRDRDLEVDTTLKSLSQQIENIRSPEGSRKNPARTCRDLKMCHSDWKSGEYWIDPNQGCNLDAIKVFCNMETGETCVYPTQPSVAQKNWYISKNPKDKRHVWFGESMTDGFQFEYGGQGSDPADVAIQLTFLRLMSTEASQNITYHCKNSVAYMDQQTGNLKKALLLQGSNEIEIRAEGNSRFTYSVTVDGCTSHTGAWGKTVIEYKTTKTSRLPIIDVAPLDVGAPDQEFGFDVGPVCFL

SEQ ID NO: 23 - protein, 831 aa, synthetic construct
MELLIHRSSAIFLTLAINALYLTSSQNITEEFYQSTCSAVSRGYLSALRTGWYTSVITIELSNIKETKCNGTDTKVKLIKQELDKYKNAVTELQLLMQNTPAVNNRACREAPQYMNYTINTTKNLNVSISKKCKCCFLGFLLGVGSAIASGIAVSKVLHLEGEVNKIKNALQLTNKAVVSLSNGVSVLTSRVLDLKNYINNQLLPMVNRQSCRISNIETVIEFQQKNSRLLEITREFSVNAGVTTPLSTYMLTNSELLSLINDMPITNDQKKLMSSNVQIVRQQSYSIMSIIKEEVLAYVVQLPIYGVIDTPCWKLHTSPLCTTNIKEGSNICLTRTDRGWYCDNAGSVSFFPQADTCKVQSNRVFCDTMNSLTLPSEVSLCNTDIFNSKYDCKIMTSKTDISSSVITSLGAIVSCYGKTKCTASNKNRGIIKTFSNGCDYVSNKGVDTVSVGNTLYYVNKLEGKNLYVKGEPIINYYDPLVFPSDEFDASISQVNEKINQSLAFIRRSDELLHNVNTGKRSNGLPGPIGPPGPRGRTGDAGPVGPPGPPGPPGPPGPPSAGFDFSFLPQPPQEKAHDGGRYYRANDANVVRDRDLEVDTTLKSLSQQIENIRSPEGSRKNPARTCRDLKMCHSDWKSGEYWIDPNQGCNLDAIKVFCNMETGETCVYPTQPSVAQKNWYISKNPKDKRHVWFGESMTDGFQFEYGGQGSDPADVAIQLTFLRLMSTEASQNITYHCKNSVAYMDQQTGNLKKALLLQGSNEIEIRAEGNSRFTYSVTVDGCTSHTGAWGKTVIEYKTTKTSRLPIIDVAPLDVGAPDQEFGFDVGPVCFL

SEQ ID NO: 24 - protein, 831 aa, synthetic construct
MELLIHRSSAIFLTLAINALYLTSSQNITEEFYQSTCSAVSRGYLSALRTGWYTSVITIELSNIKETKCNGTDTKVKLIKQELDKYKNAVTELQLLMQNTPAVNNRARREAPQYMNYTINTTKNLNVSISKKCKCCFLGFLLGVGSAIASGIAVSKVLHLEGEVNKIKNALQLTNKAVVSLSNGVSVLTSRVLDLKNYINNQLLPMVNRQSCRISNIETVIEFQQKNSRLLEITREFSVNAGVTTPLSTYMLTNSELLSLINDMPITNDQKKLMSSNVQIVRQQSYSIMSIIKEEVLAYVVQLPIYGVIDTPCWKLHTSPLCTTNIKEGSNICLTRTDRGWYCDNAGSVSFFPQADTCKVQSNRVFCDTMNSLTLPSEVSLCNTDIFNSKYDCKIMTSKTDISSSVITSLGAIVSCYGKTKCTASNKNRGIIKTFSNGCDYVSNKGVDTVSVGNTLYYVNKLEGKNLYVKGEPIINYYDPLVFPSDEFDASISQVNEKINQSLAFIRRSDELLHNVNTGKRSNGLPGPIGPPGPRGRTGDAGPVGPPGPPGPPGPPGPPSAGFDFSFLPQPPQEKAHDGGRYYRANDANVVRDRDLEVDTTLKSLSQQIENIRSPEGSRKNPARTCRDLKMCHSDWKSGEYWIDPNQGCNLDAIKVFCNMETGETCVYPTQPSVAQKNWYISKNPKDKRHVWFGESMTDGFQFEYGGQGSDPADVAIQLTFLRLMSTEASQNITYHCKNSVAYMDQQTGNLKKALLLQGSNEIEIRAEGNSRFTYSVTVDGCTSHTGAWGKTVIEYKTTKTSRLPIIDVAPLDVGAPDQEFGFDVGPVCFL

SEQ ID NO: 25 - protein, 831 aa, synthetic construct
MELLIHRSSAIFLTLAINALYLTSSQNITEEFYQSTCSAVSRGYLSALRTGWYTSVITIELSNIKETKCNGTDTKVKLIKQELDKYKNAVTELQLLMQNTPAVNNRARREAPQYMNYTINTTKNLNVSISKKRKCCFLGFLLGVGSAIASGIAVSKVLHLEGEVNKIKNALQLTNKAVVSLSNGVSVLTSRVLDLKNYINNQLLPMVNRQSCRISNIETVIEFQQKNSRLLEITREFSVNAGVTTPLSTYMLTNSELLSLINDMPITNDQKKLMSSNVQIVRQQSYSIMSIIKEEVLAYVVQLPIYGVIDTPCWKLHTSPLCTTNIKEGSNICLTRTDRGWYCDNAGSVSFFPQADTCKVQSNRVFCDTMNSLTLPSEVSLCNTDIFNSKYDCKIMTSKTDISSSVITSLGAIVSCYGKTKCTASNKNRGIIKTFSNGCDYVSNKGVDTVSVGNTLYYVNKLEGKNLYVKGEPIINYYDPLVFPSDEFDASISQVNEKINQSLAFIRRSDELLHNVNTGKRSNGLPGPIGPPGPRGRTGDAGPVGPPGPPGPPGPPGPPSAGFDFSFLPQPPQEKAHDGGRYYRANDANVVRDRDLEVDTTLKSLSQQIENIRSPEGSRKNPARTCRDLKMCHSDWKSGEYWIDPNQGCNLDAIKVFCNMETGETCVYPTQPSVAQKNWYISKNPKDKRHVWFGESMTDGFQFEYGGQGSDPADVAIQLTFLRLMSTEASQNITYHCKNSVAYMDQQTGNLKKALLLQGSNEIEIRAEGNSRFTYSVTVDGCTSHTGAWGKTVIEYKTTKTSRLPIIDVAPLDVGAPDQEFGFDVGPVCFL

SEQ ID NO: 26 - protein, 806 aa, synthetic construct
QNITEEFYQSTCSAVSRGYLSALRTGWYTSVITIELSNIKETKCNGTDTKVKLIKQELDKYKNAVTELQLLMQNTPAVNNRARREAPQYMNYTINTTKNLNVSISKKRKRRFLGFLLGVGSAIASGIAVSKVLHLEGEVNKIKNALQLTNKAVVSLSNGVSVLTSRVLDLKNYINNQLLPMVNRQSCRISNIETVIEFQQKNSRLLEITREFSVNAGVTTPLSTYMLTNSELLSLINDMPITNDQKKLMSSNVQIVRQQSYSIMSIIKEEVLAYVVQLPIYGVIDTPCWKLHTSPLCTTNIKEGSNICLTRTDRGWYCDNAGSVSFFPQADTCKVQSNRVFCDTMNSLTLPSEVSLCNTDIFNSKYDCKIMTSKTDISSSVITSLGAIVSCYGKTKCTASNKNRGIIKTFSNGCDYVSNKGVDTVSVGNTLYYVNKLEGKNLYVKGEPIINYYDPLVFPSDEFDASISQVNEKINQSLAFIRRSDELLHNVNTGKRSNGLPGPIGPPGPRGRTGDAGPVGPPGPPGPPGPPGPPSAGFDFSFLPQPPQEKAHDGGRYYRANDANVVRDRDLEVDTTLKSLSQQIENIRSPEGSRKNPARTCRDLKMCHSDWKSGEYWIDPNQGCNLDAIKVFCNMETGETCVYPTQPSVAQKNWYISKNPKDKRHVWFGESMTDGFQFEYGGQGSDPADVAIQLTFLRLMSTEASQNITYHCKNSVAYMDQQTGNLKKALLLQGSNEIEIRAEGNSRFTYSVTVDGCTSHTGAWGKTVIEYKTTKTSRLPIIDVAPLDVGAPDQEFGFDVGPVCFL

SEQ ID NO: 27 - protein, 806 aa, synthetic construct
QNITEEFYQSTCSAVSRGYLSALRTGWYTSVITIELSNIKETKCNGTDTKVKLIKQELDKYKNAVTELQLLMQNTPAVNNCACREAPQYMNYTINTTKNLNVSISKKCKCCFLGFLLGVGSAIASGIAVSKVLHLEGEVNKIKNALQLTNKAVVSLSNGVSVLTSRVLDLKNYINNQLLPMVNRQSCRISNIETVIEFQQKNSRLLEITREFSVNAGVTTPLSTYMLTNSELLSLINDMPITNDQKKLMSSNVQIVRQQSYSIMSIIKEEVLAYVVQLPIYGVIDTPCWKLHTSPLCTTNIKEGSNICLTRTDRGWYCDNAGSVSFFPQADTCKVQSNRVFCDTMNSLTLPSEVSLCNTDIFNSKYDCKIMTSKTDISSSVITSLGAIVSCYGKTKCTASNKNRGIIKTFSNGCDYVSNKGVDTVSVGNTLYYVNKLEGKNLYVKGEPIINYYDPLVFPSDEFDASISQVNEKINQSLAFIRRSDELLHNVNTGKRSNGLPGPIGPPGPRGRTGDAGPVGPPGPPGPPGPPGPPSAGFDFSFLPQPPQEKAHDGGRYYRANDANVVRDRDLEVDTTLKSLSQQIENIRSPEGSRKNPARTCRDLKMCHSDWKSGEYWIDPNQGCNLDAIKVFCNMETGETCVYPTQPSVAQKNWYISKNPKDKRHVWFGESMTDGFQFEYGGQGSDPADVAIQLTFLRLMSTEASQNITYHCKNSVAYMDQQTGNLKKALLLQGSNEIEIRAEGNSRFTYSVTVDGCTSHTGAWGKTVIEYKTTKTSRLPIIDVAPLDVGAPDQEFGFDVGPVCFL

SEQ ID NO: 28 - protein, 806 aa, synthetic construct
QNITEEFYQSTCSAVSRGYLSALRTGWYTSVITIELSNIKETKCNGTDTKVKLIKQELDKYKNAVTELQLLMQNTPAVNNRACREAPQYMNYTINTTKNLNVSISKKCKCCFLGFLLGVGSAIASGIAVSKVLHLEGEVNKIKNALQLTNKAVVSLSNGVSVLTSRVLDLKNYINNQLLPMVNRQSCRISNIETVIEFQQKNSRLLEITREFSVNAGVTTPLSTYMLTNSELLSLINDMPITNDQKKLMSSNVQIVRQQSYSIMSIIKEEVLAYVVQLPIYGVIDTPCWKLHTSPLCTTNIKEGSNICLTRTDRGWYCDNAGSVSFFPQADTCKVQSNRVFCDTMNSLTLPSEVSLCNTDIFNSKYDCKIMTSKTDISSSVITSLGAIVSCYGKTKCTASNKNRGIIKTFSNGCDYVSNKGVDTVSVGNTLYYVNKLEGKNLYVKGEPIINYYDPLVFPSDEFDASISQVNEKINQSLAFIRRSDELLHNVNTGKRSNGLPGPIGPPGPRGRTGDAGPVGPPGPPGPPGPPGPPSAGFDFSFLPQPPQEKAHDGGRYYRANDANVVRDRDLEVDTTLKSLSQQIENIRSPEGSRKNPARTCRDLKMCHSDWKSGEYWIDPNQGCNLDAIKVFCNMETGETCVYPTQPSVAQKNWYISKNPKDKRHVWFGESMTDGFQFEYGGQGSDPADVAIQLTFLRLMSTEASQNITYHCKNSVAYMDQQTGNLKKALLLQGSNEIEIRAEGNSRFTYSVTVDGCTSHTGAWGKTVIEYKTTKTSRLPIIDVAPLDVGAPDQEFGFDVGPVCFL

SEQ ID NO: 29 - protein, 806 aa, synthetic construct
QNITEEFYQSTCSAVSRGYLSALRTGWYTSVITIELSNIKETKCNGTDTKVKLIKQELDKYKNAVTELQLLMQNTPAVNNRARREAPQYMNYTINTTKNLNVSISKKCKCCFLGFLLGVGSAIASGIAVSKVLHLEGEVNKIKNALQLTNKAVVSLSNGVSVLTSRVLDLKNYINNQLLPMVNRQSCRISNIETVIEFQQKNSRLLEITREFSVNAGVTTPLSTYMLTNSELLSLINDMPITNDQKKLMSSNVQIVRQQSYSIMSIIKEEVLAYVVQLPIYGVIDTPCWKLHTSPLCTTNIKEGSNICLTRTDRGWYCDNAGSVSFFPQADTCKVQSNRVFCDTMNSLTLPSEVSLCNTDIFNSKYDCKIMTSKTDISSSVITSLGAIVSCYGKTKCTASNKNRGIIKTFSNGCDYVSNKGVDTVSVGNTLYYVNKLEGKNLYVKGEPIINYYDPLVFPSDEFDASISQVNEKINQSLAFIRRSDELLHNVNTGKRSNGLPGPIGPPGPRGRTGDAGPVGPPGPPGPPGPPGPPSAGFDFSFLPQPPQEKAHDGGRYYRANDANVVRDRDLEVDTTLKSLSQQIENIRSPEGSRKNPARTCRDLKMCHSDWKSGEYWIDPNQGCNLDAIKVFCNMETGETCVYPTQPSVAQKNWYISKNPKDKRHVWFGESMTDGFQFEYGGQGSDPADVAIQLTFLRLMSTEASQNITYHCKNSVAYMDQQTGNLKKALLLQGSNEIEIRAEGNSRFTYSVTVDGCTSHTGAWGKTVIEYKTTKTSRLPIIDVAPLDVGAPDQEFGFDVGPVCFL

SEQ ID NO: 30 - protein, 806 aa, synthetic construct
QNITEEFYQSTCSAVSRGYLSALRTGWYTSVITIELSNIKETKCNGTDTKVKLIKQELDKYKNAVTELQLLMQNTPAVNNRARREAPQYMNYTINTTKNLNVSISKKRKCCFLGFLLGVGSAIASGIAVSKVLHLEGEVNKIKNALQLTNKAVVSLSNGVSVLTSRVLDLKNYINNQLLPMVNRQSCRISNIETVIEFQQKNSRLLEITREFSVNAGVTTPLSTYMLTNSELLSLINDMPITNDQKKLMSSNVQIVRQQSYSIMSIIKEEVLAYVVQLPIYGVIDTPCWKLHTSPLCTTNIKEGSNICLTRTDRGWYCDNAGSVSFFPQADTCKVQSNRVFCDTMNSLTLPSEVSLCNTDIFNSKYDCKIMTSKTDISSSVITSLGAIVSCYGKTKCTASNKNRGIIKTFSNGCDYVSNKGVDTVSVGNTLYYVNKLEGKNLYVKGEPIINYYDPLVFPSDEFDASISQVNEKINQSLAFIRRSDELLHNVNTGKRSNGLPGPIGPPGPRGRTGDAGPVGPPGPPGPPGPPGPPSAGFDFSFLPQPPQEKAHDGGRYYRANDANVVRDRDLEVDTTLKSLSQQIENIRSPEGSRKNPARTCRDLKMCHSDWKSGEYWIDPNQGCNLDAIKVFCNMETGETCVYPTQPSVAQKNWYISKNPKDKRHVWFGESMTDGFQFEYGGQGSDPADVAIQLTFLRLMSTEASQNITYHCKNSVAYMDQQTGNLKKALLLQGSNEIEIRAEGNSRFTYSVTVDGCTSHTGAWGKTVIEYKTTKTSRLPIIDVAPLDVGAPDQEFGFDVGPVCFL

SEQ ID NO: 31 - protein, 519 aa, synthetic construct
MELLIHRSSAIFLTLAINALYLTSSQNITEEFYQSTCSAVSRGYLSALRTGWYTSVITIELSNIKETKCNGTDTKVKLIKQELDKYKNAVTELQLLMQNTPAVNNRARREAPQYMNYTINTTKNLNVSISKKRKRRFLGFLLGVGSAIASGIAVSKVLHLEGEVNKIKNALQLTNKAVVSLSNGVSVLTSRVLDLKNYINNQLLPMVNRQSCRISNIETVIEFQQKNSRLLEITREFSVNAGVTTPLSTYMLTNSELLSLINDMPITNDQKKLMSSNVQIVRQQSYSIMIIKEEVLAYVVQLPIYGVIDTPCWKLHTSPLCTTNIKEGSNICLTRTDRGWYCDNAGSVSFFPQADTCKVQSNRVFCDTMNSLTLPSEVSLCNTDIFNSKYDCKIMTSKTDISSSVITSLGAIVSCYGKTKCTASNKNRGIIKTFSNGCDYVSNKGVDTVSVGNTLYYVNKLEGKNLYVKGEPIINYYDPLVFPSDEFDASISQVNEKINQSLAFIRRSDELLHNVNTGK

SEQ ID NO: 32 - protein, 520 aa, synthetic construct
MELLIHRSSAIFLTLAINALYLTSSQNITEEFYQSTCSAVSRGYLSALRTGWYTSVITIELSNIKETKCNGTDTKVKLIKQELDKYKNAVTELQLLMQNTPAVNNCACREAPQYMNYTINTTKNLNVSISKKCKCCFLGFLLGVGSAIASGIAVSKVLHLEGEVNKIKNALQLTNKAVVSLSNGVSVLTSRVLDLKNYINNQLLPMVNRQSCRISNIETVIEFQQKNSRLLEITREFSVNAGVTTPLSTYMLTNSELLSLINDMPITNDQKKLMSSNVQIVRQQSYSIMSIIKEEVLAYVVQLPIYGVIDTPCWKLHTSPLCTTNIKEGSNICLTRTDRGWYCDNAGSVSFFPQADTCKVQSNRVFCDTMNSLTLPSEVSLCNTDIFNSKYDCKIMTSKTDISSSVITSLGAIVSCYGKTKCTASNKNRGIIKTFSNGCDYVSNKGVDTVSVGNTLYYVNKLEGKNLYVKGEPIINYYDPLVFPSDEFDASISQVNEKINQSLAFIRRSDELLHNVNTGK

SEQ ID NO: 33 - protein, 520 aa, synthetic construct
MELLIHRSSAIFLTLAINALYLTSSQNITEEFYQSTCSAVSRGYLSALRTGWYTSVITIELSNIKETKCNGTDTKVKLIKQELDKYKNAVTELQLLMQNTPAVNNRACREAPQYMNYTINTTKNLNVSISKKCKCCFLGFLLGVGSAIASGIAVSKVLHLEGEVNKIKNALQLTNKAVVSLSNGVSVLTSRVLDLKNYINNQLLPMVNRQSCRISNIETVIEFQQKNSRLLEITREFSVNAGVTTPLSTYMLTNSELLSLINDMPITNDQKKLMSSNVQIVRQQSYSIMSIIKEEVLAYVVQLPIYGVIDTPCWKLHTSPLCTTNIKEGSNICLTRTDRGWYCDNAGSVSFFPQADTCKVQSNRVFCDTMNSLTLPSEVSLCNTDIFNSKYDCKIMTSKTDISSSVITSLGAIVSCYGKTKCTASNKNRGIIKTFSNGCDYVSNKGVDTVSVGNTLYYVNKLEGKNLYVKGEPIINYYDPLVFPSDEFDASISQVNEKINQSLAFIRRSDELLHNVNTGK

SEQ ID NO: 34 - protein, 520 aa, synthetic construct
MELLIHRSSAIFLTLAINALYLTSSQNITEEFYQSTCSAVSRGYLSALRTGWYTSVITIELSNIKETKCNGTDTKVKLIKQELDKYKNAVTELQLLMQNTPAVNNRARREAPQYMNYTINTTKNLNVSISKKCKCCFLGFLLGVGSAIASGIAVSKVLHLEGEVNKIKNALQLTNKAVVSLSNGVSVLTSRVLDLKNYINNQLLPMVNRQSCRISNIETVIEFQQKNSRLLEITREFSVNAGVTTPLSTYMLTNSELLSLINDMPITNDQKKLMSSNVQIVRQQSYSIMSIIKEEVLAYVVQLPIYGVIDTPCWKLHTSPLCTTNIKEGSNICLTRTDRGWYCDNAGSVSFFPQADTCKVQSNRVFCDTMNSLTLPSEVSLCNTDIFNSKYDCKIMTSKTDISSSVITSLGAIVSCYGKTKCTASNKNRGIIKTFSNGCDYVSNKGVDTVSVGNTLYYVNKLEGKNLYVKGEPIINYYDPLVFPSDEFDASISQVNEKINQSLAFIRRSDELLHNVNTGK

SEQ ID NO: 35 - protein, 520 aa, synthetic construct
MELLIHRSSAIFLTLAINALYLTSSQNITEEFYQSTCSAVSRGYLSALRTGWYTSVITIELSNIKETKCNGTDTKVKLIKQELDKYKNAVTELQLLMQNTPAVNNRARREAPQYMNYTINTTKNLNVSISKKRKCCFLGFLLGVGSAIASGIAVSKVLHLEGEVNKIKNALQLTNKAVVSLSNGVSVLTSRVLDLKNYINNQLLPMVNRQSCRISNIETVIEFQQKNSRLLEITREFSVNAGVTTPLSTYMLTNSELLSLINDMPITNDQKKLMSSNVQIVRQQSYSIMSIIKEEVLAYVVQLPIYGVIDTPCWKLHTSPLCTTNIKEGSNICLTRTDRGWYCDNAGSVSFFPQADTCKVQSNRVFCDTMNSLTLPSEVSLCNTDIFNSKYDCKIMTSKTDISSSVITSLGAIVSCYGKTKCTASNKNRGIIKTFSNGCDYVSNKGVDTVSVGNTLYYVNKLEGKNLYVKGEPIINYYDPLVFPSDEFDASISQVNEKINQSLAFIRRSDELLHNVNTGK

SEQ ID NO: 36 - protein, 495 aa, synthetic construct
QNITEEFYQSTCSAVSRGYLSALRTGWYTSVITIELSNIKETKCNGTDTKVKLIKQELDKYKNAVTELQLLMQNTPAVNNRARREAPQYMNYTINTTKNLNVSISKKRKRRFLGFLLGVGSAIASGIAVSKVLHLEGEVNKIKNALQLTNKAVVSLSNGVSVLTSRVLDLKNYINNQLLPMVNRQSCRISNIETVIEFQQKNSRLLEITREFSVNAGVTTPLSTYMLTNSELLSLINDMPITNDQKKLMSSNVQIVRQQSYSIMSIIKEEVLAYVVQLPIYGVIDTPCWKLHTSPLCTTNIKEGSNICLTRTDRGWYCDNAGSVSFFPQADTCKVQSNRVFCDTMNSLTLPSEVSLCNTDIFNSKYDCKIMTSKTDISSSVITSLGAIVSCYGKTKCTASNKNRGIIKTFSNGCDYVSNKGVDTVSVGNTLYYVNKLEGKNLYVKGEPIINYYDPLVFPSDEFDASISQVNEKINQSLAFIRRSDELLHNVNTGK

SEQ ID NO: 37 - protein, 495 aa, synthetic construct
QNITEEFYQSTCSAVSRGYLSALRTGWYTSVITIELSNIKETKCNGTDTKVKLIKQELDKYKNAVTELQLLMQNTPAVNNCACREAPQYMNYTINTTKNLNVSISKKCKCCFLGFLLGVGSAIASGIAVSKVLHLEGEVNKIKNALQLTNKAVVSLSNGVSVLTSRVLDLKNYINNQLLPMVNRQSCRISNIETVIEFQQKNSRLLEITREFSVNAGVTTPLSTYMLTNSELLSLINDMPITNDQKKLMSSNVQIVRQQSYSIMSIIKEEVLAYVVQLPIYGVIDTPCWKLHTSPLCTTNIKEGSNICLTRTDRGWYCDNAGSVSFFPQADTCKVQSNRVFCDTMNSLTLPSEVSLCNTDIFNSKYDCKIMTSKTDISSSVITSLGAIVSCYGKTKCTASNKNRGIIKTFSNGCDYVSNKGVDTVSVGNTLYYVNKLEGKNLYVKGEPIINYYDPLVFPSDEFDASISQVNEKINQSLAFIRRSDELLHNVNTGK

SEQ ID NO: 38 - protein, 495 aa, synthetic construct
QNITEEFYQSTCSAVSRGYLSALRTGWYTSVITIELSNIKETKCNGTDTKVKLIKQELDKYKNAVTELQLLMQNTPAVNNRACREAPQYMNYTINTTKNLNVSISKKCKCCFLGFLLGVGSAIASGIAVSKVLHLEGEVNKIKNALQLTNKAVVSLSNGVSVLTSRVLDLKNYINNQLLPMVNRQSCRISNIETVIEFQQKNSRLLEITREFSVNAGVTTPLSTYMLTNSELLSLINDMPITNDQKKLMSSNVQIVRQQSYSIMSIIKEEVLAYVVQLPIYGVIDTPCWKLHTSPLCTTNIKEGSNICLTRTDRGWYCDNAGSVSFFPQADTCKVQSNRVFCDTMNSLTLPSEVSLCNTDIFNSKYDCKIMTSKTDISSSVITSLGAIVSCYGKTKCTASNKNRGIIKTFSNGCDYVSNKGVDTVSVGNTLYYVNKLEGKNLYVKGEPIINYYDPLVFPSDEFDASISQVNEKINQSLAFIRRSDELLHNVNTGK

SEQ ID NO: 39 - protein, 495 aa, synthetic construct
QNITEEFYQSTCSAVSRGYLSALRTGWYTSVITIELSNIKETKCNGTDTKVKLIKQELDKYKNAVTELQLLMQNTPAVNNRARREAPQYMNYTINTTKNLNVSISKKCKCCFLGFLLGVGSAIASGIAVSKVLHLEGEVNKIKNALQLTNKAVVSLSNGVSVLTSRVLDLKNYINNQLLPMVNRQSCRISNIETVIEFQQKNSRLLEITREFSVNAGVTTPLSTYMLTNSELLSLINDMPITNDQKKLMSSNVQIVRQQSYSIMSIIKEEVLAYVVQLPIYGVIDTPCWKLHTSPLCTTNIKEGSNICLTRTDRGWYCDNAGSVSFFPQADTCKVQSNRVFCDTMNSLTLPSEVSLCNTDIFNSKYDCKIMTSKTDISSSVITSLGAIVSCYGKTKCTASNKNRGIIKTFSNGCDYVSNKGVDTVSVGNTLYYVNKLEGKNLYVKGEPIINYYDPLVFPSDEFDASISQVNEKINQSLAFIRRSDELLHNVNTGK

SEQ ID NO: 40 - protein, 495 aa, synthetic construct
QNITEEFYQSTCSAVSRGYLSALRTGWYTSVITIELSNIKETKCNGTDTKVKLIKQELDKYKNAVTELQLLMQNTPAVNNRARREAPQYMNYTINTTKNLNVSISKKRKCCFLGFLLGVGSAIASGIAVSKVLHLEGEVNKIKNALQLTNKAVVSLSNGVSVLTSRVLDLKNYINNQLLPMVNRQSCRISNIETVIEFQQKNSRLLEITREFSVNAGVTTPLSTYMLTNSELLSLINDMPITNDQKKLMSSNVQIVRQQSYSIMSIIKEEVLAYVVQLPIYGVIDTPCWKLHTSPLCTTNIKEGSNICLTRTDRGWYCDNAGSVSFFPQADTCKVQSNRVFCDTMNSLTLPSEVSLCNTDIFNSKYDCKIMTSKTDISSSVITSLGAIVSCYGKTKCTASNKNRGIIKTFSNGCDYVSNKGVDTVSVGNTLYYVNKLEGKNLYVKGEPIINYYDPLVFPSDEFDASISQVNEKINQSLAFIRRSDELLHNVNTGK

SEQ ID NO: 41 - protein, 796 aa, synthetic construct
MELLILKANAITTILTAVTFCFASGQNITEEFYQSTCSAVSKGYLSALRTGWYTSVITIELSNIKENKCNGTDAKVKLIKQELDKYKNAVTELQLLMQSTPATNNCGGGGSAIASGVAVSKVLHLEGEVNKIKSALLSTNKAVVSLSNGVSVLTSKVLDLKNYIDKQLLPIVNKQSCSISNIATVIEFQQKNNRLLEITREFSVNAGVTTPVSTYMLTNSELLSLINDMPITNDQKKLMSNNVQIVRQQSYSIMSIIKEEVLAYVVQLPLYGVIDTPCWKLHTSPLCTTNTKEGSNICLTRTDRGWYCDNAGSVSFFPQAETCKVQSNRVFCDTMNSLTLPSEVNLCNVDIFNPKYDCKIMTSKTDVSSSVITSLGAIVSCYGKTKCTASNKNRGIIKTFSNGCDYVSNKGVDTVSVGNTLYYVNKQEGKSLYVKGEPIINFYDPLVFPSDEFDASISQVNEKINQSLAFIRKSDELLHNVNAGKRSNGLPGPIGPPGPRGRTGDAGPVGPPGPPGPPGPPGPPSAGFDFSFLPQPPQEKAHDGGRYYRANDANVVRDRDLEVDTTLKSLSQQIENIRSPEGSRKNPARTCRDLKMCHSDWKSGEYWIDPNQGCNLDAIKVFCNMETGETCVYPTQPSVAQKNWYISKNPKDKRHVWFGESMTDGFQFEYGGQGSDPADVAIQLTFLRLMSTEASQNITYHCKNSVAYMDQQTGNLKKALLLQGSNEIEIRAEGNSRFTYSVTVDGCTSHTGAWGKTVIEYKTTKTSRLPIIDVAPLDVGAPDQEFGFDVGPVCFL

SEQ ID NO: 42 - protein, 831 aa, synthetic construct
MELLILKANAITTILTAVTFCFASGQNITEEFYQSTCSAVSKGYLSALRTGWYTSVITIELSNIKENKCNGTDAKVKLIKQELDKYKNAVTELQLLMQSTPATNNCGGGELPRFMNYTLNNAKKTNVTLSKKRKRRFLGFLLGVGSAIASGVAVSKVLHLEGEVNKIKSALLSTNKAVVSLSNGVSVLTSKVLDLKNYIDKQLLPIVNKQSCSISNIATVIEFQQKNNRLLEITREFSVNAGVTTPVSTYMLTNSELLSLINDMPITNDQKKLMSNNVQIVRQQSYSIMSIIKEEVLAYVVQLPLYGVIDTPCWKLHTSPLCTTNTKEGSNICLTRTDRGWYCDNAGSVSFFPQAETCKVQSNRVFCDTMNSLTLPSEVNLCNVDIFNPKYDCKIMTSKTDVSSSVITSLGAIVSCYGKTKCTASNKNRGIIKTFSNGCDYVSNKGVDTVSVGNTLYYVNKQEGKSLYVKGEPIINFYDPLVFPSDEFDASISQVNEKINQSLAFIRKSDELLHNVNAGKRSNGLPGPIGPPGPRGRTGDAGPVGPPGPPGPPGPPGPPSAGFDFSFLPQPPQEKAHDGGRYYRANDANVVRDRDLEVDTTLKSLSQQIENIRSPEGSRKNPARTCRDLKMCHSDWKSGEYWIDPNQGCNLDAIKVFCNMETGETCVYPTQPSVAQKNWYISKNPKDKRHVWFGESMTDGFQFEYGGQGSDPADVAIQLTFLRLMSTEASQNITYHCKNSVAYMDQQTGNLKKALLLQGSNEIEIRAEGNSRFTYSVTVDGCTSHTGAWGKTVIEYKTTKTSRLPIIDVAPLDVGAPDQEFGFDVGPVCFL

SEQ ID NO: 43 - protein, 804 aa, synthetic construct
MELLILKANAITTILTAVTFCFASGQNITEEFYQSTCSAVSKGYLSALRTGWYTSVITIELSNIKENKCNGTDAKVKLIKQELDKYKNAVTELQLLMQSTPATNNCGGGFLGFLLGVGSAIASGVAVSKVLHLEGEVNKIKSALLSTNKAVVSLSNGVSVLTSKVLDLKNYIDKQLLPIVNKQSCSISNIATVIEFQQKNNRLLEITREFSVNAGVTTPVSTYMLTNSELLSLINDMPITNDQKKLMSNNVQIVRQQSYSIMSIIKEEVLAYVVQLPLYGVIDTPCWKLHTSPLCTTNTKEGSNICLTRTDRGWYCDNAGSVSFFPQAETCKVQSNRVFCDTMNSLTLPSEVNLCNVDIFNPKYDCKIMTSKTDVSSSVITSLGAIVSCYGKTKCTASNKNRGIIKTFSNGCDYVSNKGVDTVSVGNTLYYVNKQEGKSLYVKGEPIINFYDPLVFPSDEFDASISQVNEKINQSLAFIRKSDELLHNVNAGKRSNGLPGPIGPPGPRGRTGDAGPVGPPGPPGPPGPPGPPSAGFDFSFLPQPPQEKAHDGGRYYRANDANVVRDRDLEVDTTLKSLSQQIENIRSPEGSRKNPARTCRDLKMCHSDWKSGEYWIDPNQGCNLDAIKVFCNMETGETCVYPTQPSVAQKNWYISKNPKDKRHVWFGESMTDGFQFEYGGQGSDPADVAIQLTFLRLMSTEASQNITYHCKNSVAYMDQQTGNLKKALLLQGSNEIEIRAEGNSRFTYSVTVDGCTSHTGAWGKTVIEYKTTKTSRLPIIDVAPLDVGAPDQEFGFDVGPVCFL

SEQ ID NO: 44 - protein, 808 aa, synthetic construct
MELLILKANAITTILTAVTFCFASGQNITEEFYQSTCSAVSKGYLSALRTGWYTSVITIELSNIKENKCNGTDAKVKLIKQELDKYKNAVTELQLLMQSTPATNNRARRCGGGFLGFLLGVGSAIASGVAVSKVLHLEGEVNKIKSALLSTNKAVVSLSNGVSVLTSKVLDLKNYIDKQLLPIVNKQSCSISNIATVIEFQQKNNRLLEITREFSVNAGVTTPVSTYMLTNSELLSLINDMPITNDQKKLMSNNVQIVRQQSYSIMSIIKEEVLAYVVQLPLYGVIDTPCWKLHTSPLCTTNTKEGSNICLTRTDRGWYCDNAGSVSFFPQAETCKVQSNRVFCDTMNSLTLPSEVNLCNVDIFNPKYDCKIMTSKTDVSSSVITSLGAIVSCYGKTKCTASNKNRGIIKTFSNGCDYVSNKGVDTVSVGNTLYYVNKQEGKSLYVKGEPIINFYDPLVFPSDEFDASISQVNEKINQSLAFIRKSDELLHNVNAGKRSNGLPGPIGPPGPRGRTGDAGPVGPPGPPGPPGPPGPPSAGFDFSFLPQPPQEKAHDGGRYYRANDANVVRDRDLEVDTTLKSLSQQIENIRSPEGSRKNPARTCRDLKMCHSDWKSGEYWIDPNQGCNLDAIKVFCNMETGETCVYPTQPSVAQKNWYISKNPKDKRHVWFGESMTDGFQFEYGGQGSDPADVAIQLTFLRLMSTEASQNITYHCKNSVAYMDQQTGNLKKALLLQGSNEIEIRAEGNSRFTYSVTVDGCTSHTGAWGKTVIEYKTTKTSRLPIIDVAPLDVGAPDQEFGFDVGPVCFL

SEQ ID NO: 45 - protein, 771 aa, synthetic construct
QNITEEFYQSTCSAVSKGYLSALRTGWYTSVITIELSNIKENKCNGTDAKVKLIKQELDKYKNAVTELQLLMQSTPATNNCGGGGSAIASGVAVSKVLHLEGEVNKIKSALLSTNKAVVSLSNGVSVLTSKVLDLKNYIDKQLLPIVNKQSCSISNIATVIEFQQKNNRLLEITREFSVNAGVTTPVSTYMLTNSELLSLINDMPITNDQKKLMSNNVQIVRQQSYSIMSIIKEEVLAYVVQLPLYGVIDTPCWKLHTSPLCTTNTKEGSNICLTRTDRGWYCDNAGSVSFFPQAETCKVQSNRVFCDTMNSLTLPSEVNLCNVDIFNPKYDCKIMTSKTDVSSSVITSLGAIVSCYGKTKCTASNKNRGIIKTFSNGCDYVSNKGVDTVSVGNTLYYVNKQEGKSLYVKGEPIINFYDPLVFPSDEFDASISQVNEKINQSLAFIRKSDELLHNVNAGKRSNGLPGPIGPPGPRGRTGDAGPVGPPGPPGPPGPPGPPSAGFDFSFLPQPPQEKAHDGGRYYRANDANVVRDRDLEVDTTLKSLSQQIENIRSPEGSRKNPARTCRDLKMCHSDWKSGEYWIDPNQGCNLDAIKVFCNMETGETCVYPTQPSVAQKNWYISKNPKDKRHVWFGESMTDGFQFEYGGQGSDPADVAIQLTFLRLMSTEASQNITYHCKNSVAYMDQQTGNLKKALLLQGSNEIEIRAEGNSRFTYSVTVDGCTSHTGAWGKTVIEYKTTKTSRLPIIDVAPLDVGAPDQEFGFDVGPVCFL

SEQ ID NO: 46 - protein, 806 aa, synthetic construct
QNITEEFYQSTCSAVSKGYLSALRTGWYTSVITIELSNIKENKCNGTDAKVKLIKQELDKYKNAVTELQLLMQSTPATNNCGGGELPRFMNYTLNNAKKTNVTLSKKRKRRFLGFLLGVGSAIASGVAVSKVLHLEGEVNKIKSALLSTNKAVVSLSNGVSVLTSKVLDLKNYIDKQLLPIVNKQSCSISNIATVIEFQQKNNRLLEITREFSVNAGVTTPVSTYMLTNSELLSLINDMPITNDQKKLMSNNVQIVRQQSYSIMSIIKEEVLAYVVQLPLYGVIDTPCWKLHTSPLCTTNTKEGSNICLTRTDRGWYCDNAGSVSFFPQAETCKVQSNRVFCDTMNSLTLPSEVNLCNVDIFNPKYDCKIMTSKTDVSSSVITSLGAIVSCYGKTKCTASNKNRGIIKTFSNGCDYVSNKGVDTVSVGNTLYYVNKQEGKSLYVKGEPIINFYDPLVFPSDEFDASISQVNEKINQSLAFIRKSDELLHNVNAGKRSNGLPGPIGPPGPRGRTGDAGPVGPPGPPGPPGPPGPPSAGFDFSFLPQPPQEKAHDGGRYYRANDANVVRDRDLEVDTTLKSLSQQIENIRSPEGSRKNPARTCRDLKMCHSDWKSGEYWIDPNQGCNLDAIKVFCNMETGETCVYPTQPSVAQKNWYISKNPKDKRHVWFGESMTDGFQFEYGGQGSDPADVAIQLTFLRLMSTEASQNITYHCKNSVAYMDQQTGNLKKALLLQGSNEIEIRAEGNSRFTYSVTVDGCTSHTGAWGKTVIEYKTTKTSRLPIIDVAPLDVGAPDQEFGFDVGPVCFL

SEQ ID NO: 47 - protein, 779 aa, synthetic construct
QNITEEFYQSTCSAVSKGYLSALRTGWYTSVITIELSNIKENKCNGTDAKVKLIKQELDKYKNAVTELQLLMQSTPATNNCGGGFLGFLLGVGSAIASGVAVSKVLHLEGEVNKIKSALLSTNKAVVSLSNGVSVLTSKVLDLKNYIDKQLLPIVNKQSCSISNIATVIEFQQKNNRLLEITREFSVNAGVTTPVSTYMLTNSELLSLINDMPITNDQKKLMSNNVQIVRQQSYSIMSIIKEEVLAYVVQLPLYGVIDTPCWKLHTSPLCTTNTKEGSNICLTRTDRGWYCDNAGSVSFFPQAETCKVQSNRVFCDTMNSLTLPSEVNLCNVDIFNPKYDCKIMTSKTDVSSSVITSLGAIVSCYGKTKCTASNKNRGIIKTFSNGCDYVSNKGVDTVSVGNTLYYVNKQEGKSLYVKGEPIINFYDPLVFPSDEFDASISQVNEKINQSLAFIRKSDELLHNVNAGKRSNGLPGPIGPPGPRGRTGDAGPVGPPGPPGPPGPPGPPSAGFDFSFLPQPPQEKAHDGGRYYRANDANVVRDRDLEVDTTLKSLSQQIENIRSPEGSRKNPARTCRDLKMCHSDWKSGEYWIDPNQGCNLDAIKVFCNMETGETCVYPTQPSVAQKNWYISKNPKDKRHVWFGESMTDGFQFEYGGQGSDPADVAIQLTFLRLMSTEASQNITYHCKNSVAYMDQQTGNLKKALLLQGSNEIEIRAEGNSRFTYSVTVDGCTSHTGAWGKTVIEYKTTKTSRLPIIDVAPLDVGAPDQEFGFDVGPVCFL

SEQ ID NO: 48 - protein, 783 aa, synthetic construct
QNITEEFYQSTCSAVSKGYLSALRTGWYTSVITIELSNIKENKCNGTDAKVKLIKQELDKYKNAVTELQLLMQSTPATNNRARRCGGGFLGFLLGVGSAIASGVAVSKVLHLEGEVNKIKSALLSTNKAVVSLSNGVSVLTSKVLDLKNYIDKQLLPIVNKQSCSISNIATVIEFQQKNNRLLEITREFSVNAGVTTPVSTYMLTNSELLSLINDMPITNDQKKLMSNNVQIVRQQSYSIMSIIKEEVLAYVVQLPLYGVIDTPCWKLHTSPLCTTNTKEGSNICLTRTDRGWYCDNAGSVSFFPQAETCKVQSNRVFCDTMNSLTLPSEVNLCNVDIFNPKYDCKIMTSKTDVSSSVITSLGAIVSCYGKTKCTASNKNRGIIKTFSNGCDYVSNKGVDTVSVGNTLYYVNKQEGKSLYVKGEPIINFYDPLVFPSDEFDASISQVNEKINQSLAFIRKSDELLHNVNAGKRSNGLPGPIGPPGPRGRTGDAGPVGPPGPPGPPGPPGPPSAGFDFSFLPQPPQEKAHDGGRYYRANDANVVRDRDLEVDTTLKSLSQQIENIRSPEGSRKNPARTCRDLKMCHSDWKSGEYWIDPNQGCNLDAIKVFCNMETGETCVYPTQPSVAQKNWYISKNPKDKRHVWFGESMTDGFQFEYGGQGSDPADVAIQLTFLRLMSTEASQNITYHCKNSVAYMDQQTGNLKKALLLQGSNEIEIRAEGNSRFTYSVTVDGCTSHTGAWGKTVIEYKTTKTSRLPIIDVAPLDVGAPDQEFGFDVGPVCFL

SEQ ID NO: 49 - protein, 485 aa, synthetic construct
MELLILKANAITTILTAVTFCFASGQNITEEFYQSTCSAVSKGYLSALRTGWYTSVITIELSNIKENKCNGTDAKVKLIKQELDKYKNAVTELQLLMQSTPATNNCGGGGSAIASGVAVSKVLHLEGEVNKIKSALLSTNKAVVSLSNGVSVLTSKVLDLKNYIDKQLLPIVNKQSCSISNIATVIEFQQKNNRLLEITREFSVNAGVTTPVSTYMLTNSELLSLINDMPITNDQKKLMSNNVQIVRQQSYSIMSIIKEEVLAYVVQLPLYGVIDTPCWKLHTSPLCTTNTKEGSNICLTRTDRGWYCDNAGSVSFFPQAETCKVQSNRVFCDTMNSLTLPSEVNLCNVDIFNPKYDCKIMTSKTDVSSSVITSLGAIVSCYGKTKCTASNKNRGIIKTFSNGCDYVSNKGVDTVSVGNTLYYVNKQEGKSLYVKGEPIINFYDPLVFPSDEFDASISQVNEKINQSLAFIRKSDELLHNVNAGK

SEQ ID NO: 50 - protein, 460 aa, synthetic construct
QNITEEFYQSTCSAVSKGYLSALRTGWYTSVITIELSNIKENKCNGTDAKVKLIKQELDKYKNAVTELQLLMQSTPATNNCGGGGSAIASGVAVSKVLHLEGEVNKIKSALLSTNKAVVSLSNGVSVLTSKVLDLKNYIDKQLLPIVNKQSCSISNIATVIEFQQKNNRLLEITREFSVNAGVTTPVSTYMLTNSELLSLINDMPITNDQKKLMSNNVQIVRQQSYSIMSIIKEEVLAYVVQLPLYGVIDTPCWKLHTSPLCTTNTKEGSNICLTRTDRGWYCDNAGSVSFFPQAETCKVQSNRVFCDTMNSLTLPSEVNLCNVDIFNPKYDCKIMTSKTDVSSSVITSLGAIVSCYGKTKCTASNKNRGIIKTFSNGCDYVSNKGVDTVSVGNTLYYVNKQEGKSLYVKGEPIINFYDPLVFPSDEFDASISQVNEKINQSLAFIRKSDELLHNVNAGK

SEQ ID NO: 51 - protein, 105 aa, synthetic construct
MELLILKANAITTILTAVTFCFASGQNITEEFYQSTCSAVSKGYLSALRTGWYTSVITIELSNIKENKCNGTDAKVKLIKQELDKYKNAVTELQLLMQSTPATNN

SEQ ID NO: 52 - protein, 80 aa, synthetic construct
QNITEEFYQSTCSAVSKGYLSALRTGWYTSVITIELSNIKENKCNGTDAKVKLIKQELDKYKNAVTELQLLMQSTPATNN

SEQ ID NO: 53 - protein, 376 aa, synthetic construct
GSAIASGVAVSKVLHLEGEVNKIKSALLSTNKAVVSLSNGVSVLTSKVLDLKNYIDKQLLPIVNKQSCSISNIATVIEFQQKNNRLLEITREFSVNAGVTTPVSTYMLTNSELLSLINDMPITNDQKKLMSNNVQIVRQQSYSIMSIIKEEVLAYVVQLPLYGVIDTPCWKLHTSPLCTTNTKEGSNICLTRTDRGWYCDNAGSVSFFPQAETCKVQSNRVFCDTMNSLTLPSEVNLCNVDIFNPKYDCKIMTSKTDVSSSVITSLGAIVSCYGKTKCTASNKNRGIIKTFSNGCDYVSNKGVDTVSVGNTLYYVNKQEGKSLYVKGEPIINFYDPLVFPSDEFDASISQVNEKINQSLAFIRKSDELLHNVNAGK

SEQ ID NO: 54 - protein, 796 aa, synthetic construct
MELLIHRSSAIFLTLAINALYLTSSQNITEEFYQSTCSAVSRGYLSALRTGWYTSVITIELSNIKETKCNGTDTKVKLIKQELDKYKNAVTELQLLMQNTPAVNNCGGGGSAIASGIAVSKVLHLEGEVNKIKNALQLTNKAVVSLSNGVSVLTSRVLDLKNYINNQLLPMVNRQSCRISNIATVIEFQQKNSRLLEITREFSVNAGVTTPLSTYMLTNSELLSLINDMPITNDQKKLMSSNVQIVRQQSYSIMSIIKEEVLAYVVQLPIYGVIDTPCWKLHTSPLCTTNIKEGSNICLTRTDRGWYCDNAGSVSFFPQADTCKVQSNRVFCDTMNSLTLPSEVSLCNTDIFNSKYDCKIMTSKTDISSSVITSLGAIVSCYGKTKCTASNKNRGIIKTFSNGCDYVSNKGVDTVSVGNTLYYVNKLEGKNLYVKGEPIINYYDPLVFPSDEFDASISQVNEKINQSLAFIRRSDELLHNVNTGKRSNGLPGPIGPPGPRGRTGDAGPVGPPGPPGPPGPPGPPSAGFDFSFLPQPPQEKAHDGGRYYRANDANVVRDRDLEVDTTLKSLSQQIENIRSPEGSRKNPARTCRDLKMCHSDWKSGEYWIDPNQGCNLDAIKVFCNMETGETCVYPTQPSVAQKNWYISKNPKDKRHVWFGESMTDGFQFEYGGQGSDPADVAIQLTFLRLMSTEASQNITYHCKNSVAYMDQQTGNLKKALLLQGSNEIEIRAEGNSRFTYSVTVDGCTSHTGAWGKTVIEYKTTKTSRLPIIDVAPLDVGAPDQEFGFDVGPVCFL

SEQ ID NO: 55 - protein, 831 aa, synthetic construct
MELLIHRSSAIFLTLAINALYLTSSQNITEEFYQSTCSAVSRGYLSALRTGWYTSVITIELSNIKETKCNGTDTKVKLIKQELDKYKNAVTELQLLMQNTPAVNNCGGGEAPQYMNYTINTTKNLNVSISKKRKRRFLGFLLGVGSAIASGIAVSKVLHLEGEVNKIKNALQLTNKAVVSLSNGVSVLTSRVLDLKNYINNQLLPMVNRQSCRISNIETVIEFQQKNSRLLEITREFSVNAGVTTPLSTYMLTNSELLSLINDMPITNDQKKLMSSNVQIVRQQSYSIMSIIKEEVLAYVVQLPIYGVIDTPCWKLHTSPLCTTNIKEGSNICLTRTDRGWYCDNAGSVSFFPQADTCKVQSNRVFCDTMNSLTLPSEVSLCNTDIFNSKYDCKIMTSKTDISSSVITSLGAIVSCYGKTKCTASNKNRGIIKTFSNGCDYVSNKGVDTVSVGNTLYYVNKLEGKNLYVKGEPIINYYDPLVFPSDEFDASISQVNEKINQSLAFIRRSDELLHNVNTGKRSNGLPGPIGPPGPRGRTGDAGPVGPPGPPGPPGPPGPPSAGFDFSFLPQPPQEKAHDGGRYYRANDANVVRDRDLEVDTTLKSLSQQIENIRSPEGSRKNPARTCRDLKMCHSDWKSGEYWIDPNQGCNLDAIKVFCNMETGETCVYPTQPSVAQKNWYISKNPKDKRHVWFGESMTDGFQFEYGGQGSDPADVAIQLTFLRLMSTEASQNITYHCKNSVAYMDQQTGNLKKALLLQGSNEIEIRAEGNSRFTYSVTVDGCTSHTGAWGKTVIEYKTTKTSRLPIIDVAPLDVGAPDQEFGFDVGPVCFL

SEQ ID NO: 56 - protein, 804 aa, synthetic construct
MELLIHRSSAIFLTLAINALYLTSSQNITEEFYQSTCSAVSRGYLSALRTGWYTSVITIELSNIKETKCNGTDTKVKLIKQELDKYKNAVTELQLLMQNTPAVNNCGGGFLGFLLGVGSAIASGIAVSKVLHLEGEVNKIKNALQLTNKAVVSLSNGVSVLTSRVLDLKNYINNQLLPMVNRQSCRISNIATVIEFQQKNSRLLEITREFSVNAGVTTPLSTYMLTNSELLSLINDMPITNDQKKLMSSNVQIVRQQSYSIMSIIKEEVLAYVVQLPIYGVIDTPCWKLHTSPLCTTNIKEGSNICLTRTDRGWYCDNAGSVSFFPQADTCKVQSNRVFCDTMNSLTLPSEVSLCNTDIFNSKYDCKIMTSKTDISSSVITSLGAIVSCYGKTKCTASNKNRGIIKTFSNGCDYVSNKGVDTVSVGNTLYYVNKLEGKNLYVKGEPIINYYDPLVFPSDEFDASISQVNEKINQSLAFIRRSDELLHNVNTGKRSNGLPGPIGPPGPRGRTGDAGPVGPPGPPGPPGPPGPPSAGFDFSFLPQPPQEKAHDGGRYYRANDANVVRDRDLEVDTTLKSLSQQIENIRSPEGSRKNPARTCRDLKMCHSDWKSGEYWIDPNQGCNLDAIKVFCNMETGETCVYPTQPSVAQKNWYISKNPKDKRHVWFGESMTDGFQFEYGGQGSDPADVAIQLTFLRLMSTEASQNITYHCKNSVAYMDQQTGNLKKALLLQGSNEIEIRAEGNSRFTYSVTVDGCTSHTGAWGKTVIEYKTTKTSRLPIIDVAPLDVGAPDQEFGFDVGPVCFL

SEQ ID NO: 57 - protein, 808 aa, synthetic construct
MELLIHRSSAIFLTLAINALYLTSSQNITEEFYQSTCSAVSRGYLSALRTGWYTSVITIELSNIKETKCNGTDTKVKLIKQELDKYKNAVTELQLLMQNTPAVNNRARRCGGGFLGFLLGVGSAIASGIAVSKVLHLEGEVNKIKNALQLTNKAVVSLSNGVSVLTSRVLDLKNYINNQLLPMVNRQSCRISNIATVIEFQQKNSRLLEITREFSVNAGVTTPLSTYMLTNSELLSLINDMPITNDQKKLMSSNVQIVRQQSYSIMSIIKEEVLAYVVQLPIYGVIDTPCWKLHTSPLCTTNIKEGSNICLTRTDRGWYCDNAGSVSFFPQADTCKVQSNRVFCDTMNSLTLPSEVSLCNTDIFNSKYDCKIMTSKTDISSSVITSLGAIVSCYGKTKCTASNKNRGIIKTFSNGCDYVSNKGVDTVSVGNTLYYVNKLEGKNLYVKGEPIINYYDPLVFPSDEFDASISQVNEKINQSLAFIRRSDELLHNVNTGKRSNGLPGPIGPPGPRGRTGDAGPVGPPGPPGPPGPPGPPSAGFDFSFLPQPPQEKAHDGGRYYRANDANVVRDRDLEVDTTLKSLSQQIENIRSPEGSRKNPARTCRDLKMCHSDWKSGEYWIDPNQGCNLDAIKVFCNMETGETCVYPTQPSVAQKNWYISKNPKDKRHVWFGESMTDGFQFEYGGQGSDPADVAIQLTFLRLMSTEASQNITYHCKNSVAYMDQQTGNLKKALLLQGSNEIEIRAEGNSRFTYSVTVDGCTSHTGAWGKTVIEYKTTKTSRLPIIDVAPLDVGAPDQEFGFDVGPVCFL

SEQ ID NO: 58 - protein, 771 aa, synthetic construct
QNITEEFYQSTCSAVSRGYLSALRTGWYTSVITIELSNIKETKCNGTDTKVKLIKQELDKYKNAVTELQLLMQNTPAVNNCGGGGSAIASGIAVSKVLHLEGEVNKIKNALQLTNKAVVSLSNGVSVLTSRVLDLKNYINNQLLPMVNRQSCRISNIATVIEFQQKNSRLLEITREFSVNAGVTTPLSTYMLTNSELLSLINDMPITNDQKKLMSSNVQIVRQQSYSIMSIIKEEVLAYVVQLPIYGVIDTPCWKLHTSPLCTTNIKEGSNICLTRTDRGWYCDNAGSVSFFPQADTCKVQSNRVFCDTMNSLTLPSEVSLCNTDIFNSKYDCKIMTSKTDISSSVITSLGAIVSCYGKTKCTASNKNRGIIKTFSNGCDYVSNKGVDTVSVGNTLYYVNKLEGKNLYVKGEPIINYYDPLVFPSDEFDASISQVNEKINQSLAFIRRSDELLHNVNTGKRSNGLPGPIGPPGPRGRTGDAGPVGPPGPPGPPGPPGPPSAGFDFSFLPQPPQEKAHDGGRYYRANDANVVRDRDLEVDTTLKSLSQQIENIRSPEGSRKNPARTCRDLKMCHSDWKSGEYWIDPNQGCNLDAIKVFCNMETGETCVYPTQPSVAQKNWYISKNPKDKRHVWFGESMTDGFQFEYGGQGSDPADVAIQLTFLRLMSTEASQNITYHCKNSVAYMDQQTGNLKKALLLQGSNEIEIRAEGNSRFTYSVTVDGCTSHTGAWGKTVIEYKTTKTSRLPIIDVAPLDVGAPDQEFGFDVGPVCFL

SEQ ID NO: 59 - protein, 806 aa, synthetic construct
QNITEEFYQSTCSAVSRGYLSALRTGWYTSVITIELSNIKETKCNGTDTKVKLIKQELDKYKNAVTELQLLMQNTPAVNNCGGGEAPQYMNYTINTTKNLNVSISKKRKRRFLGFLLGVGSAIASGIAVSKVLHLEGEVNKIKNALQLTNKAVVSLSNGVSVLTSRVLDLKNYINNQLLPMVNRQSCRISNIATVIEFQQKNSRLLEITREFSVNAGVTTPLSTYMLTNSELLSLINDMPITNDQKKLMSSNVQIVRQQSYSIMSIIKEEVLAYVVQLPIYGVIDTPCWKLHTSPLCTTNIKEGSNICLTRTDRGWYCDNAGSVSFFPQADTCKVQSNRVFCDTMNSLTLPSEVSLCNTDIFNSKYDCKIMTSKTDISSSVITSLGAIVSCYGKTKCTASNKNRGIIKTFSNGCDYVSNKGVDTVSVGNTLYYVNKLEGKNLYVKGEPIINYYDPLVFPSDEFDASISQVNEKINQSLAFIRRSDELLHNVNTGKRSNGLPGPIGPPGPRGRTGDAGPVGPPGPPGPPGPPGPPSAGFDFSFLPQPPQEKAHDGGRYYRANDANVVRDRDLEVDTTLKSLSQQIENIRSPEGSRKNPARTCRDLKMCHSDWKSGEYWIDPNQGCNLDAIKVFCNMETGETCVYPTQPSVAQKNWYISKNPKDKRHVWFGESMTDGFQFEYGGQGSDPADVAIQLTFLRLMSTEASQNITYHCKNSVAYMDQQTGNLKKALLLQGSNEIEIRAEGNSRFTYSVTVDGCTSHTGAWGKTVIEYKTTKTSRLPIIDVAPLDVGAPDQEFGFDVGPVCFL

SEQ ID NO: 60 - protein, 779 aa, synthetic construct
QNITEEFYQSTCSAVSRGYLSALRTGWYTSVITIELSNIKETKCNGTDTKVKLIKQELDKYKNAVTELQLLMQNTPAVNNCGGGFLGFLLGVGSAIASGIAVSKVLHLEGEVNKIKNALQLTNKAVVSLSNGVSVLTSRVLDLKNYINNQLLPMVNRQSCRISNIATVIEFQQKNSRLLEITREFSVNAGVTTPLSTYMLTNSELLSLINDMPITNDQKKLMSSNVQIVRQQSYSIMSIIKEEVLAYVVQLPIYGVIDTPCWKLHTSPLCTTNIKEGSNICLTRTDRGWYCDNAGSVSFFPQADTCKVQSNRVFCDTMNSLTLPSEVSLCNTDIFNSKYDCKIMTSKTDISSSVITSLGAIVSCYGKTKCTASNKNRGIIKTFSNGCDYVSNKGVDTVSVGNTLYYVNKLEGKNLYVKGEPIINYYDPLVFPSDEFDASISQVNEKINQSLAFIRRSDELLHNVNTGKRSNGLPGPIGPPGPRGRTGDAGPVGPPGPPGPPGPPGPPSAGFDFSFLPQPPQEKAHDGGRYYRANDANVVRDRDLEVDTTLKSLSQQIENIRSPEGSRKNPARTCRDLKMCHSDWKSGEYWIDPNQGCNLDAIKVFCNMETGETCVYPTQPSVAQKNWYISKNPKDKRHVWFGESMTDGFQFEYGGQGSDPADVAIQLTFLRLMSTEASQNITYHCKNSVAYMDQQTGNLKKALLLQGSNEIEIRAEGNSRFTYSVTVDGCTSHTGAWGKTVIEYKTTKTSRLPIIDVAPLDVGAPDQEFGFDVGPVCFL

SEQ ID NO: 61 - protein, 783 aa, synthetic construct
QNITEEFYQSTCSAVSRGYLSALRTGWYTSVITIELSNIKETKCNGTDTKVKLIKQELDKYKNAVTELQLLMQNTPAVNNRARRCGGGFLGFLLGVGSAIASGIAVSKVLHLEGEVNKIKNALQLTNKAVVSLSNGVSVLTSRVLDLKNYINNQLLPMVNRQSCRISNIATVIEFQQKNSRLLEITREFSVNAGVTTPLSTYMLTNSELLSLINDMPITNDQKKLMSSNVQIVRQQSYSIMSIIKEEVLAYVVQLPIYGVIDTPCWKLHTSPLCTTNIKEGSNICLTRTDRGWYCDNAGSVSFFPQADTCKVQSNRVFCDTMNSLTLPSEVSLCNTDIFNSKYDCKIMTSKTDISSSVITSLGAIVSCYGKTKCTASNKNRGIIKTFSNGCDYVSNKGVDTVSVGNTLYYVNKLEGKNLYVKGEPIINYYDPLVFPSDEFDASISQVNEKINQSLAFIRRSDELLHNVNTGKRSNGLPGPIGPPGPRGRTGDAGPVGPPGPPGPPGPPGPPSAGFDFSFLPQPPQEKAHDGGRYYRANDANVVRDRDLEVDTTLKSLSQQIENIRSPEGSRKNPARTCRDLKMCHSDWKSGEYWIDPNQGCNLDAIKVFCNMETGETCVYPTQPSVAQKNWYISKNPKDKRHVWFGESMTDGFQFEYGGQGSDPADVAIQLTFLRLMSTEASQNITYHCKNSVAYMDQQTGNLKKALLLQGSNEIEIRAEGNSRFTYSVTVDGCTSHTGAWGKTVIEYKTTKTSRLPIIDVAPLDVGAPDQEFGFDVGPVCFL

SEQ ID NO: 62 - protein, 485 aa, synthetic construct
MELLIHRSSAIFLTLAINALYLTSSQNITEEFYQSTCSAVSRGYLSALRTGWYTSVITIELSNIKETKCNGTDTKVKLIKQELDKYKNAVTELQLLMQNTPAVNNCGGGGSAIASGIAVSKVLHLEGEVNKIKNALQLTNKAVVSLSNGVSVLTSRVLDLKNYINNQLLPMVNRQSCRISNIATVIEFQQKNSRLLEITREFSVNAGVTTPLSTYMLTNSELLSLINDMPITNDQKKLMSSNVQIVRQQSYSIMSIIKEEVLAYVVQLPIYGVIDTPCWKLHTSPLCTTNIKEGSNICLTRTDRGWYCDNAGSVSFFPQADTCKVQSNRVFCDTMNSLTLPSEVSLCNTDIFNSKYDCKIMTSKTDISSSVITSLGAIVSCYGKTKCTASNKNRGIIKTFSNGCDYVSNKGVDTVSVGNTLYYVNKLEGKNLYVKGEPIINYYDPLVFPSDEFDASISQVNEKINQSLAFIRRSDELLHNVNTGK

SEQ ID NO: 63 - protein, 460 aa, synthetic construct
QNITEEFYQSTCSAVSRGYLSALRTGWYTSVITIELSNIKETKCNGTDTKVKLIKQELDKYKNAVTELQLLMQNTPAVNNCGGGGSAIASGIAVSKVLHLEGEVNKIKNALQLTNKAVVSLSNGVSVLTSRVLDLKNYINNQLLPMVNRQSCRISNIATVIEFQQKNSRLLEITREFSVNAGVTTPLSTYMLTNSELLSLINDMPITNDQKKLMSSNVQIVRQQSYSIMSIIKEEVLAYVVQLPIYGVIDTPCWKLHTSPLCTTNIKEGSNICLTRTDRGWYCDNAGSVSFFPQADTCKVQSNRVFCDTMNSLTLPSEVSLCNTDIFNSKYDCKIMTSKTDISSSVITSLGAIVSCYGKTKCTASNKNRGIIKTFSNGCDYVSNKGVDTVSVGNTLYYVNKLEGKNLYVKGEPIINYYDPLVFPSDEFDASISQVNEKINQSLAFIRRSDELLHNVNTGK

SEQ ID NO: 64 - protein, 105 aa, synthetic construct
MELLIHRSSAIFLTLAINALYLTSSQNITEEFYQSTCSAVSRGYLSALRTGWYTSVITIELSNIKETKCNGTDTKVKLIKQELDKYKNAVTELQLLMQNTPAVNN

SEQ ID NO: 65 - protein, 80 aa, synthetic construct
QNITEEFYQSTCSAVSRGYLSALRTGWYTSVITIELSNIKETKCNGTDTKVKLIKQELDKYKNAVTELQLLMQNTPAVNN

SEQ ID NO: 66 - protein, 376 aa, synthetic construct
GSAIASGIAVSKVLHLEGEVNKIKNALQLTNKAVVSLSNGVSVLTSRVLDLKNYINNQLLPMVNRQSCRISNIATVIEFQQKNSRLLEITREFSVNAGVTTPLSTYMLTNSELLSLINDMPITNDQKKLMSSNVQIVRQQSYSIMSIIKEEVLAYVVQLPIYGVIDTPCWKLHTSPLCTTNIKEGSNICLTRTDRGWYCDNAGSVSFFPQADTCKVQSNRVFCDTMNSLTLPSEVSLCNTDIFNSKYDCKIMTSKTDISSSVITSLGAIVSCYGKTKCTASNKNRGIIKTFSNGCDYVSNKGVDTVSVGNTLYYVNKLEGKNLYVKGEPIINYYDPLVFPSDEFDASISQVNEKINQSLAFIRRSDELLHNVNTGK

SEQ ID NO: 67 - protein, 574 aa, synthetic construct
MELLILKANAITTILTAVTFCFASGQNITEEFYQSTCSAVSKGYLSALRTGWYTSVITIELSNIKENKCNGTDAKVKLIKQELDKYKNAVTELQLLMQSTPATNNRARRELPRFMNYTLNNAKKTNVTLSKKRKRRFLGFLLGVGSAIASGVAVSKVLHLEGEVNKIKSALLSTNKAVVSLSNGVSVLTSKVLDLKNYIDKQLLPIVNKQSCSISNIATVIEFQQKNNRLLEITREFSVNAGVTTPVSTYMLTNSELLSLINDMPITNDQKKLMSNNVQIVRQQSYSIMSIIKEEVLAYVVQLPLYGVIDTPCWKLHTSPLCTTNTKEGSNICLTRTDRGWYCDNAGSVSFFPQAETCKVQSNRVFCDTMNSLTLPSEVNLCNVDIFNPKYDCKIMTSKTDVSSSVITSLGAIVSCYGKTKCTASNKNRGIIKTFSNGCDYVSNKGVDTVSVGNTLYYVNKQEGKSLYVKGEPIINFYDPLVFPSDEFDASISQVNEKINQSLAFIRKSDELLHNVNAGKSTTNIMITTIIIVIIVILLSLIAVGLLLYCKARSTPVTLSKDQLSGINNIAFSN

SEQ ID NO: 68 - protein, 574 aa, synthetic construct
MELLILKANAITTILTAVTFCFASGQNITEEFYQSTCSAVSKGYLSALRTGWYTSVITIELSNIKENKCNGTDAKVKLIKQELDKYKNAVTELQLLMQSTPATNNCACRELPRFMNYTLNNAKKTNVTLSKKCKCCFLGFLLGVGSAIASGVAVSKVLHLEGEVNKIKSALLSTNKAVVSLSNGVSVLTSKVLDLKNYIDKQLLPIVNKQSCSISNIATVIEFQQKNNRLLEITREFSVNAGVTTPVSTYMLTNSELLSLINDMPITNDQKKLMSNNVQIVRQQSYSIMSIIKEEVLAYVVQLPLYGVIDTPCWKLHTSPLCTTNTKEGSNICLTRTDRGWYCDNAGSVSFFPQAETCKVQSNRVFCDTMNSLTLPSEVNLCNVDIFNPKYDCKIMTSKTDVSSSVITSLGAIVSCYGKTKCTASNKNRGIIKTFSNGCDYVSNKGVDTVSVGNTLYYVNKQEGKSLYVKGEPIINFYDPLVFPSDEFDASISQVNEKINQSLAFIRKSDELLHNVNAGKSTTNIMITTIIIVIIVILLSLIAVGLLLYCKARSTPVTLSKDQLSGINNIAFSN

SEQ ID NO: 69 - protein, 574 aa, synthetic construct
MELLIHRSSAIFLTLAINALYLTSSQNITEEFYQSTCSAVSRGYLSALRTGWYTSVITIELSNIKETKCNGTDTKVKLIKQELDKYKNAVTELQLLMQNTPAVNNRARREAPQYMNYTINTTKNLNVSISKKRKRRFLGFLLGVGSAIASGIAVSKVLHLEGEVNKIKNALQLTNKAVVSLSNGVSVLTSRVLDLKNYINNQLLPMVNRQSCRISNIETVIEFQQKNSRLLEITREFSVNAGVTTPLSTYMLTNSELLSLINDMPITNDQKKLMSSNVQIVRQQSYSIMSIIKEEVLAYVVQLPIYGVIDTPCWKLHTSPLCTTNIKEGSNICLTRTDRGWYCDNAGSVSFFPQADTCKVQSNRVFCDTMNSLTLPSEVSLCNTDIFNSKYDCKIMTSKTDISSSVITSLGAIVSCYGKTKCTASNKNRGIIKTFSNGCDYVSNKGVDTVSVGNTLYYVNKLEGKNLYVKGEPIINYYDPLVFPSDEFDASISQVNEKINQSLAFIRRSDELLHNVNTGKSTTNIMITAIIIVIIVVLLSLIAIGLLLYCKAKNTPVTLSKDQLSGINNIAFSK

SEQ ID NO: 70 - protein, 574 aa, synthetic construct
MELLIHRSSAIFLTLAINALYLTSSQNITEEFYQSTCSAVSRGYLSALRTGWYTSVITIELSNIKETKCNGTDTKVKLIKQELDKYKNAVTELQLLMQNTPAVNNCACREAPQYMNYTINTTKNLNVSISKKCKCCFLGFLLGVGSAIASGIAVSKVLHLEGEVNKIKNALQLTNKAVVSLSNGVSVLTSRVLDLKNYINNQLLPMVNRQSCRISNIETVIEFQQKNSRLLEITREFSVNAGVTTPLSTYMLTNSELLSLINDMPITNDQKKLMSSNVQIVRQQSYSIMSIIKEEVLAYVVQLPIYGVIDTPCWKLHTSPLCTTNIKEGSNICLTRTDRGWYCDNAGSVSFFPQADTCKVQSNRVFCDTMNSLTLPSEVSLCNTDIFNSKYDCKIMTSKTDISSSVITSLGAIVSCYGKTKCTASNKNRGIIKTFSNGCDYVSNKGVDTVSVGNTLYYVNKLEGKNLYVKGEPIINYYDPLVFPSDEFDASISQVNEKINQSLAFIRRSDELLHNVNTGKSTTNIMITAIIIVIIVVLLSLIAIGLLLYCKAKNTPVTLSKDQLSGINNIAFSK

SEQ ID NO: 71 - protein, 25 aa, synthetic construct
MELLILKANAITTILTAVTFCFASG

SEQ ID NO: 72 - protein, 25 aa, synthetic construct
MELLIHRSSAIFLTLAINALYLTSS

SEQ ID NO: 73 - protein, 84 aa, synthetic construct
QNITEEFYQSTCSAVSKGYLSALRTGWYTSVITIELSNIKENKCNGTDAKVKLIKQELDKYKNAVTELQLLMQSTPATNNRARR

SEQ ID NO: 74 - protein, 84 aa, synthetic construct
QNITEEFYQSTCSAVSKGYLSALRTGWYTSVITIELSNIKENKCNGTDAKVKLIKQELDKYKNAVTELQLLMQSTPATNNCACR

SEQ ID NO: 75 - protein, 4 aa, synthetic construct
RARR

SEQ ID NO: 76 - protein, 4 aa, synthetic construct
CARR

SEQ ID NO: 77 - protein, 4 aa, synthetic construct
RACR

SEQ ID NO: 78 - protein, 4 aa, synthetic construct
CACR

SEQ ID NO: 79 - protein, 27 aa, synthetic construct
ELPRFMNYTLNNAKKTNVTLSKKRKRR

SEQ ID NO: 80 - protein, 27 aa, unidentified
ELPRFMNYTLNNAKKTNVTLSKKCKCC

SEQ ID NO: 81 - protein, 27 aa, synthetic construct
EAPQYMNYTINTTKNLNVSISKKRKRR

SEQ ID NO: 82 - protein, 27 aa, synthetic construct
EAPQYMNYTINTTKNLNVSISKKCKCC

SEQ ID NO: 83 - protein, 6 aa, synthetic construct
KKRKRR

SEQ ID NO: 84 - protein, 6 aa, synthetic construct
KKCKRR

SEQ ID NO: 85 - protein, 6 aa, synthetic construct
KKRKCR

SEQ ID NO: 86 - protein, 6 aa, synthetic construct
KKRKRC

SEQ ID NO: 87 - protein, 6 aa, synthetic construct
KKCKCR

SEQ ID NO: 88 - protein, 6 aa, synthetic construct
KKCKRC

SEQ ID NO: 89 - protein, 6 aa, synthetic construct
KKRKCC

SEQ ID NO: 90 - protein, 6 aa, synthetic construct
KKCKCC

SEQ ID NO: 91 - protein, 19 aa, synthetic construct
FLGFLLGVGSAIASGVAVS

SEQ ID NO: 92 - protein, 19 aa, synthetic construct
FLGFLLGVGSAIASGIAVS

SEQ ID NO: 93 - protein, 8 aa, synthetic construct
FLGFLLGV

SEQ ID NO: 94 - protein, 388 aa, synthetic construct
FLGFLLGVGSAIASGVAVSKVLHLEGEVNKIKSALLSTNKAVVSLSNGVSVLTSKVLDLKNYIDKQLLPIVNKQSCSISNIATVIEFQQKNNRLLEITREFSVNAGVTTPVSTYMLTNSELLSLINDMPITNDQKKLMSNNVQIVRQQSYSIMSIIKEEVLAYVVQLPLYGVIDTPCWKLHTSPLCTTNTKEGSNICLTRTDRGWYCDNAGSVSFFPQAETCKVQSNRVFCDTMNSLTLPSEVNLCNVDIFNPKYDCKIMTSKTDVSSSVITSLGAIVSCYGKTKCTASNKNRGIIKTFSNGCDYVSNKGVDTVSVGNTLYYVNKQEGKSLYVKGEPIINFYDPLVFPSDEFDASISQVNEKINQSLAFIRKSDELLHNVNAGKSTIN

SEQ ID NO: 95 - protein, 384 aa, synthetic construct
FLGFLLGVGSAIASGVAVSKVLHLEGEVNKIKSALLSTNKAVVSLSNGVSVLTSKVLDLKNYIDKQLLPIVNKQSCSISNIATVIEFQQKNNRLLEITREFSVNAGVTTPVSTYMLTNSELLSLINDMPITNDQKKLMSNNVQIVRQQSYSIMSIIKEEVLAYVVQLPLYGVIDTPCWKLHTSPLCTTNTKEGSNICLTRTDRGWYCDNAGSVSFFPQAETCKVQSNRVFCDTMNSLTLPSEVNLCNVDIFNPKYDCKIMTSKTDVSSSVITSLGAIVSCYGKTKCTASNKNRGIIKTFSNGCDYVSNKGVDTVSVGNTLYYVNKQEGKSLYVKGEPIINFYDPLVFPSDEFDASISQVNEKINQSLAFIRKSDELLHNVNAGK

SEQ ID NO: 96 - protein, 388 aa, synthetic construct
FLGFLLGVGSAIASGIAVSKVLHLEGEVNKIKNALQLTNKAVVSLSNGVSVLTSRVLDLKNYINNQLLPMVNRQSCRISNIETVIEFQQKNSRLLEITREFSVNAGVTTPLSTYMLTNSELLSLINDMPITNDQKKLMSSNVQIVRQQSYSIMSIIKEEVLAYVVQLPIYGVIDTPCWKLHTSPLCTTNIKEGSNICLTRTDRGWYCDNAGSVSFFPQADTCKVQSNRVFCDTMNSLTLPSEVSLCNTDIFNSKYDCKIMTSKTDISSSVITSLGAIVSCYGKTKCTASNKNRGIIKTFSNGCDYVSNKGVDTVSVGNTLYYVNKLEGKNLYVKGEPIINYYDPLVFPSDEFDASISQVNEKINQSLAFIRRSDELLHNVNTGKSTTN

SEQ ID NO: 97 - protein, 384 aa, synthetic construct
FLGFLLGVGSAIASGIAVSKVLHLEGEVNKIKNALQLTNKAVVSLSNGVSVLTSRVLDLKNYINNQLLPMVNRQSCRISNIETVIEFQQKNSRLLEITREFSVNAGVTTPLSTYMLTNSELLSLINDMPITNDQKKLMSSNVQIVRQQSYSIMSIIKEEVLAYVVQLPIYGVIDTPCWKLHTSPLCTTNIKEGSNICLTRTDRGWYCDNAGSVSFFPQADTCKVQSNRVFCDTMNSLTLPSEVSLCNTDIFNSKYDCKIMTSKTDISSSVITSLGAIVSCYGKTKCTASNKNRGIIKTFSNGCDYVSNKGVDTVSVGNTLYYVNKLEGKNLYVKGEPIINYYDPLVFPSDEFDASISQVNEKINQSLAFIRRSDELLHNVNTGK

SEQ ID NO: 98 - protein, 26 aa, synthetic construct
IMITTIIIVIIVILLSLIAVGLLLYC

SEQ ID NO: 99 - protein, 24 aa, synthetic construct
KARSTPVTLSKDQLSGINNIAFSN

SEQ ID NO: 100 - protein, 26 aa, synthetic construct
IMITAIIIVIIVVLLSLIAIGLLLYC

SEQ ID NO: 101 - protein, 24 aa, synthetic construct
KAKNTPVTLSKDQLSGINNIAFSK

SEQ ID NO: 102 - protein, 4 aa, synthetic construct
CGGG

SEQ ID NO: 103 - protein, 244 aa, synthetic construct
ANVVRDRDLEVDTTLKSLSQQIENIRSPEGSRKNPARTCRDLKMCHSDWKSGEYWIDPNQGCNLDAIKVFCNMETGETCVYPTQPSVAQKNWYISKNPKDKRHVWFGESMTDGFQFEYGGQGSDPADVAIQLTFLRLMSTEASQNITYHCKNSVAYMDQQTGNLKKALLLQGSNEIEIRAEGNSRFTYSVTVDGCTSHTGAWGKTVIEYKTTKTSRLPIIDVAPLDVGAPDQEFGFDVGPVCFL

SEQ ID NO: 104 - protein, 246 aa, synthetic construct
RSANVVRDRDLEVDTTLKSLSQQIENIRSPEGSRKNPARTCRDLKMCHSDWKSGEYWIDPNQGCNLDAIKVFCNMETGETCVYPTQPSVAQKNWYISKNPKDKRHVWFGESMTDGFQFEYGGQGSDPADVAIQLTFLRLMSTEASQNITYHCKNSVAYMDQQTGNLKKALLLQGSNEIEIRAEGNSRFTYSVTVDGCTSHTGAWGKTVIEYKTTKTSRLPIIDVAPLDVGAPDQEFGFDVGPVCFL

SEQ ID NO: 105 - protein, 309 aa, synthetic construct
NGLPGPIGPPGPRGRTGDAGPVGPPGPPGPPGPPGPPSAGFDFSFLPQPPQEKAHDGGRYYRANDANVVRDRDLEVDTTLKSLSQQIENIRSPEGSRKNPARTCRDLKMCHSDWKSGEYWIDPNQGCNLDAIKVFCNMETGETCVYPTQPSVAQKNWYISKNPKDKRHVWFGESMTDGFQFEYGGQGSDPADVAIQLTFLRLMSTEASQNITYHCKNSVAYMDQQTGNLKKALLLQGSNEIEIRAEGNSRFTYSVTVDGCTSHTGAWGKTVIEYKTTKTSRLPIIDVAPLDVGAPDQEFGFDVGPVCFL

SEQ ID NO: 106 - protein, 309 aa, synthetic construct
NGLPGPIGPPGPRGRTGDAGPVGPPGPPGPPGPPGPPSAGFDFSFLPQPPQEKAHDGGRYYRNDDANVVRDRDLEVDTTLKSLSQQIENIRSPEGSRKNPARTCRDLKMCHSDWKSGEYWIDPNQGCNLDAIKVFCNMETGETCVYPTQPSVAQKNWYISKNPKDKRHVWFGESMTDGFQFEYGGQGSDPADVAIQLTFLRLMSTEASQNITYHCKNSVAYMDQQTGNLKKALLLQGSNEIEIRAEGNSRFTYSVTVDGCTSHTGAWGKTVIEYKTTKTSRLPIIDVAPLDVGAPDQEFGFDVGPVCFL

SEQ ID NO: 107 - protein, 311 aa, synthetic construct
RSNGLPGPIGPPGPRGRTGDAGPVGPPGPPGPPGPPGPPSAGFDFSFLPQPPQEKAHDGGRYYRANDANVVRDRDLEVDTTLKSLSQQIENIRSPEGSRKNPARTCRDLKMCHSDWKSGEYWIDPNQGCNLDAIKVFCNMETGETCVYPTQPSVAQKNWYISKNPKDKRHVWFGESMTDGFQFEYGGQGSDPADVAIQLTFLRLMSTEASQNITYHCKNSVAYMDQQTGNLKKALLLQGSNEIEIRAEGNSRFTYSVTVDGCTSHTGAWGKTVIEYKTTKTSRLPIIDVAPLDVGAPDQEFGFDVGPVCFL

SEQ ID NO: 108 - protein, 311 aa, synthetic construct
GSNGLPGPIGPPGPRGRTGDAGPVGPPGPPGPPGPPGPPSAGFDFSFLPQPPQEKAHDGGRYYRANDANVVRDRDLEVDTTLKSLSQQIENIRSPEGSRKNPARTCRDLKMCHSDWKSGEYWIDPNQGCNLDAIKVFCNMETGETCVYPTQPSVAQKNWYISKNPKDKRHVWFGESMTDGFQFEYGGQGSDPADVAIQLTFLRLMSTEASQNITYHCKNSVAYMDQQTGNLKKALLLQGSNEIEIRAEGNSRFTYSVTVDGCTSHTGAWGKTVIEYKTTKTSRLPIIDVAPLDVGAPDQEFGFDVGPVCFL

SEQ ID NO: 109 - protein, 244 aa, synthetic construct
ANVVRDRDLEVDTTLKSLSQQIENIRSPEGSRKNPARTCRDLKMCHSDWKSGEYWIDPNQGCNLDAIKVFCNMETGETCVYPTQPSVAQKNWYISKNPKDKRHVWFGESMTDGFQFEYGGQGSDPADVAIQLTFLRLMSTEASQNITYHCKNSVAYMDQQTGNLKKALLLKGSNEIEIRAEGNSRFTYSVTVDGCTSHTGAWGKTVIEYKTTKSSRLPIIDVAPLDVGAPDQEFGFDVGPVCFL

SEQ ID NO: 110 - protein, 246 aa, synthetic construct
RSANVVRDRDLEVDTTLKSLSQQIENIRSPEGSRKNPARTCRDLKMCHSDWKSGEYWIDPNQGCNLDAIKVFCNMETGETCVYPTQPSVAQKNWYISKNPKDKRHVWFGESMTDGFQFEYGGQGSDPADVAIQLTFLRLMSTEASQNITYHCKNSVAYMDQQTGNLKKALLLKGSNEIEIRAEGNSRFTYSVTVDGCTSHTGAWGKTVIEYKTTKSSRLPIIDVAPLDVGAPDQEFGFDVGPVCFL

SEQ ID NO: 111 - protein, 309 aa, synthetic construct
NGLPGPIGPPGPRGRTGDAGPVGPPGPPGPPGPPGPPSAGFDFSFLPQPPQEKAHDGGRYYRANDANVVRDRDLEVDTTLKSLSQQIENIRSPEGSRKNPARTCRDLKMCHSDWKSGEYWIDPNQGCNLDAIKVFCNMETGETCVYPTQPSVAQKNWYISKNPKDKRHVWFGESMTDGFQFEYGGQGSDPADVAIQLTFLRLMSTEASQNITYHCKNSVAYMDQQTGNLKKALLLKGSNEIEIRAEGNSRFTYSVTVDGCTSHTGAWGKTVIEYKTTKSSRLPIIDVAPLDVGAPDQEFGFDVGPVCFL

SEQ ID NO: 112 - protein, 309 aa, synthetic construct
NGLPGPIGPPGPRGRTGDAGPVGPPGPPGPPGPPGPPSAGFDFSFLPQPPQEKAHDGGRYYRNDDANVVRDRDLEVDTTLKSLSQQIENIRSPEGSRKNPARTCRDLKMCHSDWKSGEYWIDPNQGCNLDAIKVFCNMETGETCVYPTQPSVAQKNWYISKNPKDKRHVWFGESMTDGFQFEYGGQGSDPADVAIQLTFLRLMSTEASQNITYHCKNSVAYMDQQTGNLKKALLLKGSNEIEIRAEGNSRFTYSVTVDGCTSHTGAWGKTVIEYKTTKSSRLPIIDVAPLDVGAPDQEFGFDVGPVCFL

SEQ ID NO: 113 - protein, 311 aa, synthetic construct
RSNGLPGPIGPPGPRGRTGDAGPVGPPGPPGPPGPPGPPSAGFDFSFLPQPPQEKAHDGGRYYRANDANVVRDRDLEVDTTLKSLSQQIENIRSPEGSRKNPARTCRDLKMCHSDWKSGEYWIDPNQGCNLDAIKVFCNMETGETCVYPTQPSVAQKNWYISKNPKDKRHVWFGESMTDGFQFEYGGQGSDPADVAIQLTFLRLMSTEASQNITYHCKNSVAYMDQQTGNLKKALLLKGSNEIEIRAEGNSRFTYSVTVDGCTSHTGAWGKTVIEYKTTKSSRLPIIDVAPLDVGAPDQEFGFDVGPVCFL

SEQ ID NO: 114 - protein, 311 aa, synthetic construct
GSNGLPGPIGPPGPRGRTGDAGPVGPPGPPGPPGPPGPPSAGFDFSFLPQPPQEKAHDGGRYYRANDANVVRDRDLEVDTTLKSLSQQIENIRSPEGSRKNPARTCRDLKMCHSDWKSGEYWIDPNQGCNLDAIKVFCNMETGETCVYPTQPSVAQKNWYISKNPKDKRHVWFGESMTDGFQFEYGGQGSDPADVAIQLTFLRLMSTEASQNITYHCKNSVAYMDQQTGNLKKALLLKGSNEIEIRAEGNSRFTYSVTVDGCTSHTGAWGKTVIEYKTTKSSRLPIIDVAPLDVGAPDQEFGFDVGPVCFL

SEQ ID NO: 115 - protein, 234 aa, synthetic construct
DEIMTSLKSVNGQIESLISPDGSRKNPARNCRDLKFCHPELKSGEYWVDPNQGCKLDAIKVFCNMETGETCISANPLNVPRKHWWTDSSAEKKHVWFGESMDGGFQFSYGNPELPEDVLDVQLAFLRLLSSRASQNITYHCKNSIAYMDQASGNVKKALKLMGSNEGEFKAEGNSKFTYTVLEDGCTKHTGEWSKTVFEYRTRKAVRLPIVDIAPYDIGGPDQEFGVDVGPVCF

SEQ ID NO: 116 - protein, 244 aa, synthetic construct
EPMDFKINTDEIMTSLKSVNGQIESLISPDGSRKNPARNCRDLKFCHPELKSGEYWVDPNQGCKLDAIKVFCNMETGETCISANPLNVPRKHWWTDSSAEKKHVWFGESMDGGFQFSYGNPELPEDVLDVQLAFLRLLSSRASQNITYHCKNSIAYMDQASGNVKKALKLMGSNEGEFKAEGNSKFTYTVLEDGCTKHTGEWSKTVFEYRTRKAVRLPIVDIAPYDIGGPDQEFGVDVGPVCFL

SEQ ID NO: 117 - protein, 245 aa, synthetic construct
SEPMDFKINTDEIMTSLKSVNGQIESLISPDGSRKNPARNCRDLKFCHPELKSGEYWVDPNQGCKLDAIKVFCNMETGETCISANPLNVPRKHWWTDSSAEKKHVWFGESMDGGFQFSYGNPELPEDVLDVQLAFLRLLSSRASQNITYHCKNSIAYMDQASGNVKKALKLMGSNEGEFKAEGNSKFTYTVLEDGCTKHTGEWSKTVFEYRTRKAVRLPIVDIAPYDIGGPDQEFGVDVGPVCFL

SEQ ID NO: 118 - protein, 246 aa, synthetic construct
RSEPMDFKINTDEIMTSLKSVNGQIESLISPDGSRKNPARNCRDLKFCHPELKSGEYWVDPNQGCKLDAIKVFCNMETGETCISANPLNVPRKHWWTDSSAEKKHVWFGESMDGGFQFSYGNPELPEDVLDVQLAFLRLLSSRASQNITYHCKNSIAYMDQASGNVKKALKLMGSNEGEFKAEGNSKFTYTVLEDGCTKHTGEWSKTVFEYRTRKAVRLPIVDIAPYDIGGPDQEFGVDVGPVCFL

SEQ ID NO: 119 - protein, 84 aa, synthetic construct
QNITEEFYQSTCSAVSRGYLSALRTGWYTSVITIELSNIKETKCNGTDTKVKLIKQELDKYKNAVTELQLLMQNTPAVNNRARR

SEQ ID NO: 120 - protein, 84 aa, synthetic construct
QNITEEFYQSTCSAVSRGYLSALRTGWYTSVITIELSNIKETKCNGTDTKVKLIKQELDKYKNAVTELQLLMQNTPAVNNCACR

SEQ ID NO: 121 - protein, 4 aa, synthetic construct
RSAN

SEQ ID NO: 122 - protein, 4 aa, synthetic construct
DDAN

SEQ ID NO: 123 - protein, 6 aa, synthetic construct
RADDAN

SEQ ID NO: 124 - protein, 6 aa, synthetic construct
RANDAN

SEQ ID NO: 125 - protein, 6 aa, synthetic construct
RNDDAN

SEQ ID NO: 126 - protein, 8 aa, synthetic construct
FLGFLLGV

SEQ ID NO: 127 - protein, 4 aa, synthetic construct
FLGF

SEQ ID NO: 128 - protein, 5 aa, synthetic construct
FLGFL

SEQ ID NO: 129 - protein, 6 aa, synthetic construct
FLGFLL

SEQ ID NO: 130 - protein, 7 aa, synthetic construct
FLGFLLG

SEQ ID NO: 131 - protein, 8 aa, synthetic construct
FLGFLLGV

SEQ ID NO: 132 - DNA, 22 bp, synthetic construct
  source 1..22: mol_type = other DNA
tccatggacgttcctgagcgtt

SEQ ID NO: 133 - DNA, 20 bp, synthetic construct
  source 1..20: mol_type = other DNA
ggtgcatcgatgcagggggg

SEQ ID NO: 134 - DNA, 22 bp, synthetic construct
  source 1..22: mol_type = other DNA
tcgtcgttcgaacgacgttgat

SEQ ID NO: 135 - DNA, 23 bp, synthetic construct
  source 1..23: mol_type = other DNA
tcgtcgacgatcggcgcgcgccg

SEQ ID NO: 136 - DNA, 24 bp, synthetic construct
  source 1..24: mol_type = other DNA
tcgtcgttttgtcgttttgtcgtt

SEQ ID NO: 137 - DNA, 22 bp, synthetic construct
  source 1..22: mol_type = other DNA
tgactgtgaacgttcgagatga

SEQ ID NO: 138 - protein, 4 aa, synthetic construct
CGGG

SEQ ID NO: 139 - protein, 831 aa, synthetic construct
MELLILKANAITTILTAVTFCFASGQNITEEFYQSTCSAVSKGYLSALRTGWYTSVITIELSNIKENKCNGTDAKVKLIKQELDKYKNAVTELQLLMQSTPATNNAAARELPRFMNYTLNNAKKTNVTLSKKAKAAFLGFLLGVGSAIASGVAVSKVLHLEGEVNKIKSALLSTNKAVVSLSNGVSVLTSKVLDLKNYIDKQLLPIVNKQSCSISNIATVIEFQQKNNRLLEITREFSVNAGVTTPVSTYMLTNSELLSLINDMPITNDQKKLMSNNVQIVRQQSYSIMSIIKEEVLAYVVQLPLYGVIDTPCWKLHTSPLCTTNTKEGSNICLTRTDRGWYCDNAGSVSFFPQAETCKVQSNRVFCDTMNSLTLPSEVNLCNVDIFNPKYDCKIMTSKTDVSSSVITSLGAIVSCYGKTKCTASNKNRGIIKTFSNGCDYVSNKGVDTVSVGNTLYYVNKQEGKSLYVKGEPIINFYDPLVFPSDEFDASISQVNEKINQSLAFIRKSDELLHNVNAGKRSNGLPGPIGPPGPRGRTGDAGPVGPPGPPGPPGPPGPPSAGFDFSFLPQPPQEKAHDGGRYYRANDANVVRDRDLEVDTTLKSLSQQIENIRSPEGSRKNPARTCRDLKMCHSDWKSGEYWIDPNQGCNLDAIKVFCNMETGETCVYPTQPSVAQKNWYISKNPKDKRHVWFGESMTDGFQFEYGGQGSDPADVAIQLTFLRLMSTEASQNITYHCKNSVAYMDQQTGNLKKALLLQGSNEIEIRAEGNSRFTYSVTVDGCTSHTGAWGKTVIEYKTTKTSRLPIIDVAPLDVGAPDQEFGFDVGPVCFL

SEQ ID NO: 140 - protein, 831 aa, synthetic construct
MELLILKANAITTILTAVTFCFASGQNITEEFYQSTCSAVSKGYLSALRTGWYTSVITIELSNIKENKCNGTDAKVKLIKQELDKYKNAVTELQLLMQSTPATNNTATRELPRFMNYTLNNAKKTNVTLSKKTKTTFLGFLLGVGSAIASGVAVSKVLHLEGEVNKIKSALLSTNKAVVSLSNGVSVLTSKVLDLKNYIDKQLLPIVNKQSCSISNIATVIEFQQKNNRLLEITREFSVNAGVTTPVSTYMLTNSELLSLINDMPITNDQKKLMSNNVQIVRQQSYSIMSIIKEEVLAYVVQLPLYGVIDTPCWKLHTSPLCTTNTKEGSNICLTRTDRGWYCDNAGSVSFFPQAETCKVQSNRVFCDTMNSLTLPSEVNLCNVDIFNPKYDCKIMTSKTDVSSSVITSLGAIVSCYGKTKCTASNKNRGIIKTFSNGCDYVSNKGVDTVSVGNTLYYVNKQEGKSLYVKGEPIINFYDPLVFPSDEFDASISQVNEKINQSLAFIRKSDELLHNVNAGKRSNGLPGPIGPPGPRGRTGDAGPVGPPGPPGPPGPPGPPSAGFDFSFLPQPPQEKAHDGGRYYRANDANVVRDRDLEVDTTLKSLSQQIENIRSPEGSRKNPARTCRDLKMCHSDWKSGEYWIDPNQGCNLDAIKVFCNMETGETCVYPTQPSVAQKNWYISKNPKDKRHVWFGESMTDGFQFEYGGQGSDPADVAIQLTFLRLMSTEASQNITYHCKNSVAYMDQQTGNLKKALLLQGSNEIEIRAEGNSRFTYSVTVDGCTSHTGAWGKTVIEYKTTKTSRLPIIDVAPLDVGAPDQEFGFDVGPVCFL

SEQ ID NO: 141 - protein, 831 aa, synthetic construct
MELLILKANAITTILTAVTFCFASGQNITEEFYQSTCSAVSKGYLSALRTGWYTSVITIELSNIKENKCNGTDAKVKLIKQELDKYKNAVTELQLLMQSTPATNNYAYRELPRFMNYTLNNAKKTNVTLSKKYKYYFLGFLLGVGSAIASGVAVSKVLHLEGEVNKIKSALLSTNKAVVSLSNGVSVLTSKVLDLKNYIDKQLLPIVNKQSCSISNIATVIEFQQKNNRLLEITREFSVNAGVTTPVSTYMLTNSELLSLINDMPITNDQKKLMSNNVQIVRQQSYSIMSIIKEEVLAYVVQLPLYGVIDTPCWKLHTSPLCTTNTKEGSNICLTRTDRGWYCDNAGSVSFFPQAETCKVQSNRVFCDTMNSLTLPSEVNLCNVDIFNPKYDCKIMTSKTDVSSSVITSLGAIVSCYGKTKCTASNKNRGIIKTFSNGCDYVSNKGVDTVSVGNTLYYVNKQEGKSLYVKGEPIINFYDPLVFPSDEFDASISQVNEKINQSLAFIRKSDELLHNVNAGKRSNGLPGPIGPPGPRGRTGDAGPVGPPGPPGPPGPPGPPSAGFDFSFLPQPPQEKAHDGGRYYRANDANVVRDRDLEVDTTLKSLSQQIENIRSPEGSRKNPARTCRDLKMCHSDWKSGEYWIDPNQGCNLDAIKVFCNMETGETCVYPTQPSVAQKNWYISKNPKDKRHVWFGESMTDGFQFEYGGQGSDPADVAIQLTFLRLMSTEASQNITYHCKNSVAYMDQQTGNLKKALLLQGSNEIEIRAEGNSRFTYSVTVDGCTSHTGAWGKTVIEYKTTKTSRLPIIDVAPLDVGAPDQEFGFDVGPVCFL

SEQ ID NO: 142 - protein, 831 aa, synthetic construct
MELLILKANAITTILTAVTFCFASGQNITEEFYQSTCSAVSKGYLSALRTGWYTSVITIELSNIKENKCNGTDAKVKLIKQELDKYKNAVTELQLLMQSTPATNNGAGRELPRFMNYTLNNAKKTNVTLSKKGKGGFLGFLLGVGSAIASGVAVSKVLHLEGEVNKIKSALLSTNKAVVSLSNGVSVLTSKVLDLKNYIDKQLLPIVNKQSCSISNIATVIEFQQKNNRLLEITREFSVNAGVTTPVSTYMLTNSELLSLINDMPITNDQKKLMSNNVQIVRQQSYSIMSIIKEEVLAYVVQLPLYGVIDTPCWKLHTSPLCTTNTKEGSNICLTRTDRGWYCDNAGSVSFFPQAETCKVQSNRVFCDTMNSLTLPSEVNLCNVDIFNPKYDCKIMTSKTDVSSSVITSLGAIVSCYGKTKCTASNKNRGIIKTFSNGCDYVSNKGVDTVSVGNTLYYVNKQEGKSLYVKGEPIINFYDPLVFPSDEFDASISQVNEKINQSLAFIRKSDELLHNVNAGKRSNGLPGPIGPPGPRGRTGDAGPVGPPGPPGPPGPPGPPSAGFDFSFLPQPPQEKAHDGGRYYRANDANVVRDRDLEVDTTLKSLSQQIENIRSPEGSRKNPARTCRDLKMCHSDWKSGEYWIDPNQGCNLDAIKVFCNMETGETCVYPTQPSVAQKNWYISKNPKDKRHVWFGESMTDGFQFEYGGQGSDPADVAIQLTFLRLMSTEASQNITYHCKNSVAYMDQQTGNLKKALLLQGSNEIEIRAEGNSRFTYSVTVDGCTSHTGAWGKTVIEYKTTKTSRLPIIDVAPLDVGAPDQEFGFDVGPVCFL

SEQ ID NO: 143 - protein, 831 aa, synthetic construct
MELLILKANAITTILTAVTFCFASGQNITEEFYQSTCSAVSKGYLSALRTGWYTSVITIELSNIKENKCNGTDAKVKLIKQELDKYKNAVTELQLLMQSTPATNNSASRELPRFMNYTLNNAKKTNVTLSKKSKSSFLGFLLGVGSAIASGVAVSKVLHLEGEVNKIKSALLSTNKAVVSLSNGVSVLTSKVLDLKNYIDKQLLPIVNKQSCSISNIATVIEFQQKNNRLLEITREFSVNAGVTTPVSTYMLTNSELLSLINDMPITNDQKKLMSNNVQIVRQQSYSIMSIIKEEVLAYVVQLPLYGVIDTPCWKLHTSPLCTTNTKEGSNICLTRTDRGWYCDNAGSVSFFPQAETCKVQSNRVFCDTMNSLTLPSEVNLCNVDIFNPKYDCKIMTSKTDVSSSVITSLGAIVSCYGKTKCTASNKNRGIIKTFSNGCDYVSNKGVDTVSVGNTLYYVNKQEGKSLYVKGEPIINFYDPLVFPSDEFDASISQVNEKINQSLAFIRKSDELLHNVNAGKRSNGLPGPIGPPGPRGRTGDAGPVGPPGPPGPPGPPGPPSAGFDFSFLPQPPQEKAHDGGRYYRANDANVVRDRDLEVDTTLKSLSQQIENIRSPEGSRKNPARTCRDLKMCHSDWKSGEYWIDPNQGCNLDAIKVFCNMETGETCVYPTQPSVAQKNWYISKNPKDKRHVWFGESMTDGFQFEYGGQGSDPADVAIQLTFLRLMSTEASQNITYHCKNSVAYMDQQTGNLKKALLLQGSNEIEIRAEGNSRFTYSVTVDGCTSHTGAWGKTVIEYKTTKTSRLPIIDVAPLDVGAPDQEFGFDVGPVCFL

SEQ ID NO: 144 - protein, 831 aa, synthetic construct
MELLIHRSSAIFLTLAINALYLTSSQNITEEFYQSTCSAVSRGYLSALRTGWYTSVITIELSNIKETKCNGTDTKVKLIKQELDKYKNAVTELQLLMQNTPAVNNAAAREAPQYMNYTINTTKNLNVSISKKAKAAFLGFLLGVGSAIASGIAVSKVLHLEGEVNKIKNALQLTNKAVVSLSNGVSVLTSRVLDLKNYINNQLLPMVNRQSCRISNIETVIEFQQKNSRLLEITREFSVNAGVTTPLSTYMLTNSELLSLINDMPITNDQKKLMSSNVQIVRQQSYSIMSIIKEEVLAYVVQLPIYGVIDTPCWKLHTSPLCTTNIKEGSNICLTRTDRGWYCDNAGSVSFFPQADTCKVQSNRVFCDTMNSLTLPSEVSLCNTDIFNSKYDCKIMTSKTDISSSVITSLGAIVSCYGKTKCTASNKNRGIIKTFSNGCDYVSNKGVDTVSVGNTLYYVNKLEGKNLYVKGEPIINYYDPLVFPSDEFDASISQVNEKINQSLAFIRRSDELLHNVNTGKRSNGLPGPIGPPGPRGRTGDAGPVGPPGPPGPPGPPGPPSAGFDFSFLPQPPQEKAHDGGRYYRANDANVVRDRDLEVDTTLKSLSQQIENIRSPEGSRKNPARTCRDLKMCHSDWKSGEYWIDPNQGCNLDAIKVFCNMETGETCVYPTQPSVAQKNWYISKNPKDKRHVWFGESMTDGFQFEYGGQGSDPADVAIQLTFLRLMSTEASQNITYHCKNSVAYMDQQTGNLKKALLLQGSNEIEIRAEGNSRFTYSVTVDGCTSHTGAWGKTVIEYKTTKTSRLPIIDVAPLDVGAPDQEFGFDVGPVCFL

SEQ ID NO: 145 - protein, 831 aa, synthetic construct
MELLIHRSSAIFLTLAINALYLTSSQNITEEFYQSTCSAVSRGYLSALRTGWYTSVITIELSNIKETKCNGTDTKVKLIKQELDKYKNAVTELQLLMQNTPAVNNTATREAPQYMNYTINTTKNLNVSISKKTKTTFLGFLLGVGSAIASGIAVSKVLHLEGEVNKIKNALQLTNKAVVSLSNGVSVLTSRVLDLKNYINNQLLPMVNRQSCRISNIETVIEFQQKNSRLLEITREFSVNAGVTTPLSTYMLTNSELLSLINDMPITNDQKKLMSSNVQIVRQQSYSIMSIIKEEVLAYVVQLPIYGVIDTPCWKLHTSPLCTTNIKEGSNICLTRTDRGWYCDNAGSVSFFPQADTCKVQSNRVFCDTMNSLTLPSEVSLCNTDIFNSKYDCKIMTSKTDISSSVITSLGAIVSCYGKTKCTASNKNRGIIKTFSNGCDYVSNKGVDTVSVGNTLYYVNKLEGKNLYVKGEPIINYYDPLVFPSDEFDASISQVNEKINQSLAFIRRSDELLHNVNTGKRSNGLPGPIGPPGPRGRTGDAGPVGPPGPPGPPGPPGPPSAGFDFSFLPQPPQEKAHDGGRYYRANDANVVRDRDLEVDTTLKSLSQQIENIRSPEGSRKNPARTCRDLKMCHSDWKSGEYWIDPNQGCNLDAIKVFCNMETGETCVYPTQPSVAQKNWYISKNPKDKRHVWFGESMTDGFQFEYGGQGSDPADVAIQLTFLRLMSTEASQNITYHCKNSVAYMDQQTGNLKKALLLQGSNEIEIRAEGNSRFTYSVTVDGCTSHTGAWGKTVIEYKTTKTSRLPIIDVAPLDVGAPDQEFGFDVGPVCFL

SEQ ID NO: 146 - protein, 831 aa, synthetic construct
MELLIHRSSAIFLTLAINALYLTSSQNITEEFYQSTCSAVSRGYLSALRTGWYTSVITIELSNIKETKCNGTDTKVKLIKQELDKYKNAVTELQLLMQNTPAVNNYAYREAPQYMNYTINTTKNLNVSISKKYKYYFLGFLLGVGSAIASGIAVSKVLHLEGEVNKIKNALQLTNKAVVSLSNGVSVLTSRVLDLKNYINNQLLPMVNRQSCRISNIETVIEFQQKNSRLLEITREFSVNAGVTTPLSTYMLTNSELLSLINDMPITNDQKKLMSSNVQIVRQQSYSIMSIIKEEVLAYVVQLPIYGVIDTPCWKLHTSPLCTTNIKEGSNICLTRTDRGWYCDNAGSVSFFPQADTCKVQSNRVFCDTMNSLTLPSEVSLCNTDIFNSKYDCKIMTSKTDISSSVITSLGAIVSCYGKTKCTASNKNRGIIKTFSNGCDYVSNKGVDTVSVGNTLYYVNKLEGKNLYVKGEPIINYYDPLVFPSDEFDASISQVNEKINQSLAFIRRSDELLHNVNTGKRSNGLPGPIGPPGPRGRTGDAGPVGPPGPPGPPGPPGPPSAGFDFSFLPQPPQEKAHDGGRYYRANDANVVRDRDLEVDTTLKSLSQQIENIRSPEGSRKNPARTCRDLKMCHSDWKSGEYWIDPNQGCNLDAIKVFCNMETGETCVYPTQPSVAQKNWYISKNPKDKRHVWFGESMTDGFQFEYGGQGSDPADVAIQLTFLRLMSTEASQNITYHCKNSVAYMDQQTGNLKKALLLQGSNEIEIRAEGNSRFTYSVTVDGCTSHTGAWGKTVIEYKTTKTSRLPIIDVAPLDVGAPDQEFGFDVGPVCFL

SEQ ID NO: 147 - protein, 831 aa, synthetic construct
MELLIHRSSAIFLTLAINALYLTSSQNITEEFYQSTCSAVSRGYLSALRTGWYTSVITIELSNIKETKCNGTDTKVKLIKQELDKYKNAVTELQLLMQNTPAVNNGAGREAPQYMNYTINTTKNLNVSISKKGKGGFLGFLLGVGSAIASGIAVSKVLHLEGEVNKIKNALQLTNKAVVSLSNGVSVLTSRVLDLKNYINNQLLPMVNRQSCRISNIETVIEFQQKNSRLLEITREFSVNAGVTTPLSTYMLTNSELLSLINDMPITNDQKKLMSSNVQIVRQQSYSIMSIIKEEVLAYVVQLPIYGVIDTPCWKLHTSPLCTTNIKEGSNICLTRTDRGWYCDNAGSVSFFPQADTCKVQSNRVFCDTMNSLTLPSEVSLCNTDIFNSKYDCKIMTSKTDISSSVITSLGAIVSCYGKTKCTASNKNRGIIKTFSNGCDYVSNKGVDTVSVGNTLYYVNKLEGKNLYVKGEPIINYYDPLVFPSDEFDASISQVNEKINQSLAFIRRSDELLHNVNTGKRSNGLPGPIGPPGPRGRTGDAGPVGPPGPPGPPGPPGPPSAGFDFSFLPQPPQEKAHDGGRYYRANDANVVRDRDLEVDTTLKSLSQQIENIRSPEGSRKNPARTCRDLKMCHSDWKSGEYWIDPNQGCNLDAIKVFCNMETGETCVYPTQPSVAQKNWYISKNPKDKRHVWFGESMTDGFQFEYGGQGSDPADVAIQLTFLRLMSTEASQNITYHCKNSVAYMDQQTGNLKKALLLQGSNEIEIRAEGNSRFTYSVTVDGCTSHTGAWGKTVIEYKTTKTSRLPIIDVAPLDVGAPDQEFGFDVGPVCFL

SEQ ID NO: 148 - protein, 831 aa, synthetic construct
MELLIHRSSAIFLTLAINALYLTSSQNITEEFYQSTCSAVSRGYLSALRTGWYTSVITIELSNIKETKCNGTDTKVKLIKQELDKYKNAVTELQLLMQNTPAVNNSASREAPQYMNYTINTTKNLNVSISKKSKSSFLGFLLGVGSAIASGIAVSKVLHLEGEVNKIKNALQLTNKAVVSLSNGVSVLTSRVLDLKNYINNQLLPMVNRQSCRISNIETVIEFQQKNSRLLEITREFSVNAGVTTPLSTYMLTNSELLSLINDMPITNDQKKLMSSNVQIVRQQSYSIMSIIKEEVLAYVVQLPIYGVIDTPCWKLHTSPLCTTNIKEGSNICLTRTDRGWYCDNAGSVSFFPQADTCKVQSNRVFCDTMNSLTLPSEVSLCNTDIFNSKYDCKIMTSKTDISSSVITSLGAIVSCYGKTKCTASNKNRGIIKTFSNGCDYVSNKGVDTVSVGNTLYYVNKLEGKNLYVKGEPIINYYDPLVFPSDEFDASISQVNEKINQSLAFIRRSDELLHNVNTGKRSNGLPGPIGPPGPRGRTGDAGPVGPPGPPGPPGPPGPPSAGFDFSFLPQPPQEKAHDGGRYYRANDANVVRDRDLEVDTTLKSLSQQIENIRSPEGSRKNPARTCRDLKMCHSDWKSGEYWIDPNQGCNLDAIKVFCNMETGETCVYPTQPSVAQKNWYISKNPKDKRHVWFGESMTDGFQFEYGGQGSDPADVAIQLTFLRLMSTEASQNITYHCKNSVAYMDQQTGNLKKALLLQGSNEIEIRAEGNSRFTYSVTVDGCTSHTGAWGKTVIEYKTTKTSRLPIIDVAPLDVGAPDQEFGFDVGPVCFL